European Patent Application EP 4 636 087 A1, published October 22, 2025. Title: Anti-GPA33 antibody and use thereof. Applicant: 国立大学法人 鹿児島大学. The sequence listing filed with the application follows.

SEQUENCE LISTING (353 sequences)

SEQ ID NO: 1 - protein, 6 aa, synthetic construct
  source 1..6: note = 2RC9 VL CDR1 / 2RC28 VL CDR1
QSISSY

SEQ ID NO: 2 - protein, 9 aa, synthetic construct
  source 1..9: note = 2RC9 VL CDR3
QQSYRTPYT

SEQ ID NO: 3 - protein, 8 aa, synthetic construct
  source 1..8: note = 2RC9 VH CDR1
GFTFSNYN

SEQ ID NO: 4 - protein, 8 aa, synthetic construct
  source 1..8: note = 2RC9 VH CDR2 / 2RC17 VH CDR2
ISSSGDFM

SEQ ID NO: 5 - protein, 11 aa, synthetic construct
  source 1..11: note = 2RC9 VH CDR3 / 2RC17 VH CDR3
AREGPGTPFDY

SEQ ID NO: 6 - protein, 6 aa, synthetic construct
  source 1..6: note = 2RC17 VL CDR1
QSISSF

SEQ ID NO: 7 - protein, 9 aa, synthetic construct
  source 1..9: note = 2RC17 VL CDR3
QQSHNTPYT

SEQ ID NO: 8 - protein, 8 aa, synthetic construct
  source 1..8: note = 2RC17 VH CDR1
GFTFSSYN

SEQ ID NO: 9 - protein, 8 aa, synthetic construct
  source 1..8: note = 2RC28 VL CDR3
QQSYNTWT

SEQ ID NO: 10 - protein, 8 aa, synthetic construct
  source 1..8: note = 2RC28 VH CDR1
GFTFSSYS

SEQ ID NO: 11 - protein, 8 aa, synthetic construct
  source 1..8: note = 2RC28 VH CDR2
ISRDSTVI

SEQ ID NO: 12 - protein, 11 aa, synthetic construct
  source 1..11: note = 2RC28 VH CDR3
AREGVAGAFDI

SEQ ID NO: 13 - protein, 107 aa, synthetic construct
  source 1..107: note = 2RC9 VL
AIQMTQSPSSLSASVGDRVTITCRASQSISSYLNWYQQKPGKAPKLLIYAASSLQSGVPSRFSGSGSGTDFTLTISSLQPEDFATYYCQQSYRTPYTFGQGTKVEIK

SEQ ID NO: 14 - protein, 118 aa, synthetic construct
  source 1..118: note = 2RC9 VH
QVQLVQSGGGLVKPGGSLRLSCAASGFTFSNYNMNWVRQAPGKGLEWVSSISSSGDFMYYADSVKGRFTISRDDAKNSLYLQMNSLRAEDTAVYYCAREGPGTPFDYWGQGTLVTVSS

SEQ ID NO: 15 - protein, 107 aa, synthetic construct
  source 1..107: note = 2RC17 VL
AIQLTQSPSSLSASVGDRVTITCRASQSISSFLNWYQHKPGKAPKLLIYVASSLQSGVPSRFSGSGSGTDFTLTISSLQPEDFATYYCQQSHNTPYTFGQGTKLEIK

SEQ ID NO: 16 - protein, 118 aa, synthetic construct
  source 1..118: note = 2RC17 VH
QMQLVQSGGGLVKPGGSLRLSCAASGFTFSSYNMNWVRQAPGKGLEWVSSISSSGDFMYYADSVKGRFTISRDNAKNSLYLQMSSLRAEDTAVYYCAREGPGTPFDYWGQGTLVTVSS

SEQ ID NO: 17 - protein, 106 aa, synthetic construct
  source 1..106: note = 2RC28 VL
AIQLTQSPSSLSASVGDRVTITCRASQSISSYLNWYQQKPGKAPKLLIYIASSLQSGVPSRFSGSGSGTDFTLTISSLQPEDFATYYCQQSYNTWTFGQGTKVEIK

SEQ ID NO: 18 - protein, 118 aa, synthetic construct
  source 1..118: note = 2RC28 VH
EVQLVESGGGLVKPGGSLRLSCAASGFTFSSYSMNWVRQAPGKGLEWVSSISRDSTYIYYADSVKGRFTISRDNAKNSLYLQMNSLRAEDTAVYYCAREGVAGAFDIWGQGTMVTVSS

SEQ ID NO: 19 - protein, 210 aa, synthetic construct
  source 1..210: note = Fc
PSVFLFPPKPKDTLMISRTPEVTCVVVDVSHEDPEVKFNWYVDGVEVHNAKTKPREEQYNSTYRVVSVLTVLHQDWLNGKEYKCAVSNKALPASIEKTISKAKGQPREPQVYTLPPSREEMTKNQVSLTCLVKGFYPSDIAVEWESNGQPENNYKTTPPVLDSDGSFFLYSKLTVDKSRWQQGNVFSCSVMHEALHNHYTQKSLSLSPGK

SEQ ID NO: 20 - protein, 240 aa, synthetic construct
  source 1..240: note = 2RC9
QVQLVQSGGGLVKPGGSLRLSCAASGFTFSNYNMNWVRQAPGKGLEWVSSISSSGDFMYYADSVKGRFTISRDDAKNSLYLQMNSLRAEDTAVYYCAREGPGTPFDYWGQGTLVTVSSGGGGSGGGGSGSTGSAIQMTQSPSSLSASVGDRVTITCRASQSISSYLNWYQQKPGKAPKLLIYAASSLQSGVPSRFSGSGSGTDFTLTISSLQPEDFATYYCQQSYRTPYTFGQGTKVEIK

SEQ ID NO: 21 - protein, 240 aa, synthetic construct
  source 1..240: note = 2RC17
QMQLVQSGGGLVKPGGSLRLSCAASGFTFSSYNMNWVRQAPGKGLEWVSSISSSGDFMYYADSVKGRFTISRDNAKNSLYLQMSSLRAEDTAVYYCAREGPGTPFDYWGQGTLVTVSSGGGGSGGGGSGSTGSAIQLTQSPSSLSASVGDRVTITCRASQSISSFLNWYQHKPGKAPKLLIYVASSLQSGVPSRFSGSGSGTDFTLTISSLQPEDFATYYCQQSHNTPYTFGQGTKLEIK

SEQ ID NO: 22 - protein, 239 aa, synthetic construct
  source 1..239: note = 2RC28
EVQLVESGGGLVKPGGSLRLSCAASGFTFSSYSMNWVRQAPGKGLEWVSSISRDSTYIYYADSVKGRFTISRDNAKNSLYLQMNSLRAEDTAVYYCAREGVAGAFDIWGQGTMVTVSSGGGGSGGGGSGSTGSAIQLTQSPSSLSASVGDRVTITCRASQSISSYLNWYQQKPGKAPKLLIYIASSLQSGVPSRFSGSGSGTDFTLTISSLQPEDFATYYCQQSYNTWTFGQGTKVEIK

SEQ ID NO: 23 - protein, 269 aa, synthetic construct
  source 1..269: note = 2RC9-Cys
QVQLVQSGGGLVKPGGSLRLSCAASGFTFSNYNMNWVRQAPGKGLEWVSSISSSGDFMYYADSVKGRFTISRDDAKNSLYLQMNSLRAEDTAVYYCAREGPGTPFDYWGQGTLVTVSSGGGGSGGGGSGSTGSAIQMTQSPSSLSASVGDRVTITCRASQSISSYLNWYQQKPGKAPKLLIYAASSLQSGVPSRFSGSGSGTDFTLTISSLQPEDFATYYCQQSYRTPYTFGQGTKVEIKAACTSAHHHHHHGAAEQKLISEEDLNGAA

SEQ ID NO: 24 - protein, 269 aa, synthetic construct
  source 1..269: note = 2RC17-Cys
QMQLVQSGGGLVKPGGSLRLSCAASGFTFSSYNMNWVRQAPGKGLEWVSSISSSGDFMYYADSVKGRFTISRDNAKNSLYLQMSSLRAEDTAVYYCAREGPGTPFDYWGQGTLVTVSSGGGGSGGGGSGSTGSAIQLTQSPSSLSASVGDRVTITCRASQSISSFLNWYQHKPGKAPKLLIYVASSLQSGVPSRFSGSGSGTDFTLTISSLQPEDFATYYCQQSHNTPYTFGQGTKLEIKAACTSAHHHHHHGAAEQKLISEEDLNGAA

SEQ ID NO: 25 - protein, 268 aa, synthetic construct
  source 1..268: note = 2RC28-Cys
EVQLVESGGGLVKPGGSLRLSCAASGFTFSSYSMNWVRQAPGKGLEWVSSISRDSTYIYYADSVKGRFTISRDNAKNSLYLQMNSLRAEDTAVYYCAREGVAGAFDIWGQGTMVTVSSGGGGSGGGGSGSTGSAIQLTQSPSSLSASVGDRVTITCRASQSISSYLNWYQQKPGKAPKLLIYIASSLQSGVPSRFSGSGSGTDFTLTISSLQPEDFATYYCQQSYNTWTFGQGTKVEIKAACTSAHHHHHHGAAEQKLISEEDLNGAA

SEQ ID NO: 26 - protein, 471 aa, synthetic construct
  source 1..471: note = GPA2RC9-Fc
QVQLVQSGGGLVKPGGSLRLSCAASGFTFSNYNMNWVRQAPGKGLEWVSSISSSGDFMYYADSVKGRFTISRDDAKNSLYLQMNSLRAEDTAVYYCAREGPGTPFDYWGQGTLVTVSSGGGGSGGGGSGSTGSAIQMTQSPSSLSASVGDRVTITCRASQSISSYLNWYQQKPGKAPKLLIYAASSLQSGVPSRFSGSGSGTDFTLTISSLQPEDFATYYCQQSYRTPYTFGQGTKVEIKPKSSDKTHTCPPCPAPEAEGAPSVFLFPPKPKDTLMISRTPEVTCVVVDVSHEDPEVKFNWYVDGVEVHNAKTKPREEQYNSTYRVVSVLTVLHQDWLNGKEYKCAVSNKALPASIEKTISKAKGQPREPQVYTLPPSREEMTKNQVSLTCLVKGFYPSDIAVEWESNGQPENNYKTTPPVLDSDGSFFLYSKLTVDKSRWQQGNVFSCSVMHEALHNHYTQKSLSLSPGK

SEQ ID NO: 27 - protein, 471 aa, synthetic construct
  source 1..471: note = GPA2RC17-Fc
QMQLVQSGGGLVKPGGSLRLSCAASGFTFSSYNMNWVRQAPGKGLEWVSSISSSGDFMYYADSVKGRFTISRDNAKNSLYLQMSSLRAEDTAVYYCAREGPGTPFDYWGQGTLVTVSSGGGGSGGGGSGSTGSAIQLTQSPSSLSASVGDRVTITCRASQSISSFLNWYQHKPGKAPKLLIYVASSLQSGVPSRFSGSGSGTDFTLTISSLQPEDFATYYCQQSHNTPYTFGQGTKLEIKPKSSDKTHTCPPCPAPEAEGAPSVFLFPPKPKDTLMISRTPEVTCVVVDVSHEDPEVKFNWYVDGVEVHNAKTKPREEQYNSTYRVVSVLTVLHQDWLNGKEYKCAVSNKALPASIEKTISKAKGQPREPQVYTLPPSREEMTKNQVSLTCLVKGFYPSDIAVEWESNGQPENNYKTTPPVLDSDGSFFLYSKLTVDKSRWQQGNVFSCSVMHEALHNHYTQKSLSLSPGK

SEQ ID NO: 28 - protein, 470 aa, synthetic construct
  source 1..470: note = GPA2RC28-Fc
EVQLVESGGGLVKPGGSLRLSCAASGFTFSSYSMNWVRQAPGKGLEWVSSISRDSTYIYYADSVKGRFTISRDNAKNSLYLQMNSLRAEDTAVYYCAREGVAGAFDIWGQGTMVTVSSGGGGSGGGGSGSTGSAIQLTQSPSSLSASVGDRVTITCRASQSISSYLNWYQQKPGKAPKLLIYIASSLQSGVPSRFSGSGSGTDFTLTISSLQPEDFATYYCQQSYNTWTFGQGTKVEIKPKSSDKTHTCPPCPAPEAEGAPSVFLFPPKPKDTLMISRTPEVTCVVVDVSHEDPEVKFNWYVDGVEVHNAKTKPREEQYNSTYRVVSVLTVLHQDWLNGKEYKCAVSNKALPASIEKTISKAKGQPREPQVYTLPPSREEMTKNQVSLTCLVKGFYPSDIAVEWESNGQPENNYKTTPPVLDSDGSFFLYSKLTVDKSRWQQGNVFSCSVMHEALHNHYTQKSLSLSPGK

SEQ ID NO: 29 - protein, 13 aa, synthetic construct
  REGION 1..13: note = Fc binding peptide
  SITE 6: note = MISC_FEATURE - X is K, C, D, E, R, V, F, L, 2-Aminooctanedioic acid, Dpr, Orn,AcOrn, AcDab, Dab, Nle, Nva, Tle, Ala(t-Bu), or Cha
DCAYHXGELVWCT

SEQ ID NO: 30 - protein, 17 aa, synthetic construct
  REGION 1..17: note = IgG binding peptide
  SITE 8: note = MISC_FEATURE - X is K, C, D, E, R, V, F, L, 2-Aminooctanedioic acid, Dpr, Orn,AcOrn, AcDab, Dab, Nle, Nva, Tle, Ala(t-Bu), or Cha
GPDCAYHXGELVWCTFH

SEQ ID NO: 31 - protein, 13 aa, synthetic construct
  REGION 1..13: note = IgG binding peptide
  SITE 6: note = MISC_FEATURE - X is K, C, D, E, R, V, F, L, 2-Aminooctanedioic acid, Dpr, Orn,AcOrn, AcDab, Dab, Nle, Nva, Tle, Ala(t-Bu), or Cha
RCAYHXGELVWCS

SEQ ID NO: 32 - protein, 17 aa, synthetic construct
  REGION 1..17: note = IgG binding peptide
  SITE 8: note = MISC_FEATURE - X is K, C, D, E, R, V, F, L, 2-Aminooctanedioic acid, Dpr, Orn,AcOrn, AcDab, Dab, Nle, Nva, Tle, Ala(t-Bu), or Cha
GPRCAYHXGELVWCSFH

SEQ ID NO: 33 - protein, 17 aa, synthetic construct
  REGION 1..17: note = IgG binding peptide
  SITE 8: note = MISC_FEATURE - X is K, C, D, E, R, V, F, L, 2-Aminooctanedioic acid, Dpr, Orn,AcOrn, AcDab, Dab, Nle, Nva, Tle, Ala(t-Bu), or Cha
SPDCAYHXGELVWCTFH

SEQ ID NO: 34 - protein, 17 aa, synthetic construct
  REGION 1..17: note = IgG binding peptide
  SITE 8: note = MISC_FEATURE - X is K, C, D, E, R, V, F, L, 2-Aminooctanedioic acid, Dpr, Orn,AcOrn, AcDab, Dab, Nle, Nva, Tle, Ala(t-Bu), or Cha
GDDCAYHXGELVWCTFH

SEQ ID NO: 35 - protein, 17 aa, synthetic construct
  REGION 1..17: note = IgG binding peptide
  SITE 8: note = MISC_FEATURE - X is K, C, D, E, R, V, F, L, 2-Aminooctanedioic acid, Dpr, Orn,AcOrn, AcDab, Dab, Nle, Nva, Tle, Ala(t-Bu), or Cha
GPSCAYHXGELVWCTFH

SEQ ID NO: 36 - protein, 17 aa, synthetic construct
  REGION 1..17: note = IgG binding peptide
  SITE 8: note = MISC_FEATURE - X is K, C, D, E, R, V, F, L, 2-Aminooctanedioic acid, Dpr, Orn,AcOrn, AcDab, Dab, Nle, Nva, Tle, Ala(t-Bu), or Cha
GPDCAYHXGELVWCSFH

SEQ ID NO: 37 - protein, 17 aa, synthetic construct
  REGION 1..17: note = IgG binding peptide
  SITE 8: note = MISC_FEATURE - X is K, C, D, E, R, V, F, L, 2-Aminooctanedioic acid, Dpr, Orn,AcOrn, AcDab, Dab, Nle, Nva, Tle, Ala(t-Bu), or Cha
GPDCAYHXGELVWCTHH

SEQ ID NO: 38 - protein, 17 aa, synthetic construct
  REGION 1..17: note = IgG binding peptide
  SITE 8: note = MISC_FEATURE - X is K, C, D, E, R, V, F, L, 2-Aminooctanedioic acid, Dpr, Orn,AcOrn, AcDab, Dab, Nle, Nva, Tle, Ala(t-Bu), or Cha
GPDCAYHXGELVWCTFY

SEQ ID NO: 39 - protein, 17 aa, synthetic construct
  REGION 1..17: note = IgG binding peptide
  SITE 8: note = MISC_FEATURE - X is K,C, D, E, R, V, F, L, 2-Aminooctanedioic acid, Dpr, Orn,AcOrn, AcDab, Dab, Nle, Nva, Tle, Ala(t-Bu), or Cha
SPDCAYHXGELVWCTFY

SEQ ID NO: 40 - protein, 17 aa, synthetic construct
  REGION 1..17: note = IgG binding peptide
  SITE 8: note = MISC_FEATURE - X is K, C, D, E, R, V, F, L, 2-Aminooctanedioic acid, Dpr, Orn,AcOrn, AcDab, Dab, Nle, Nva, Tle, Ala(t-Bu), or Cha
SDDCAYHXGELVWCTFY

SEQ ID NO: 41 - protein, 17 aa, synthetic construct
  REGION 1..17: note = IgG binding peptide
  SITE 8: note = MISC_FEATURE - X is K, C, D, E, R, V, F, L, 2-Aminooctanedioic acid, Dpr, Orn,AcOrn, AcDab, Dab, Nle, Nva, Tle, Ala(t-Bu), or Cha
RGNCAYHXGQLVWCTYH

SEQ ID NO: 42 - protein, 17 aa, synthetic construct
  REGION 1..17: note = IgG binding peptide
  SITE 2: note = MISC_FEATURE - X is homocysteine
  SITE 8: note = MISC_FEATURE - X is K, C, D, E, R, V, F, L, 2-Aminooctanedioic acid, Dpr, Orn,AcOrn, AcDab, Dab, Nle, Nva, Tle, Ala(t-Bu), or Cha
  SITE 16: note = MISC_FEATURE - X is homocysteine
GXDCAYHXGELVWCTXH

SEQ ID NO: 43 - protein, 19 aa, synthetic construct
  REGION 1..19: note = IgG binding peptide
  SITE 10: note = MISC_FEATURE - X is K, C, D, E, R, V, F, L, 2-Aminooctanedioic acid, Dpr, Orn,AcOrn, AcDab, Dab, Nle, Nva, Tle, Ala(t-Bu), or Cha
RRGPDCAYHXGELVWCTFH

SEQ ID NO: 44 - protein, 13 aa, synthetic construct
  REGION 1..13: note = IgG binding peptide
  SITE 6: note = MISC_FEATURE - X is K, C, D, E, R, V, F, L, 2-Aminooctanedioic acid, Dpr, Orn,AcOrn, AcDab, Dab, Nle, Nva, Tle, Ala(t-Bu), or Cha
DCTYHXGNLVWCT

SEQ ID NO: 45 - protein, 13 aa, synthetic construct
  REGION 1..13: note = IgG binding peptide
  SITE 6: note = MISC_FEATURE - X is K, C, D, E, R, V, F, L, 2-Aminooctanedioic acid, Dpr, Orn,AcOrn, AcDab, Dab, Nle, Nva, Tle, Ala(t-Bu), or Cha
DCAYHXGNLVWCT

SEQ ID NO: 46 - protein, 13 aa, synthetic construct
  REGION 1..13: note = IgG binding peptide
  SITE 6: note = MISC_FEATURE - X is K, C, D, E, R, V, F, L, 2-Aminooctanedioic acid, Dpr, Orn,AcOrn, AcDab, Dab, Nle, Nva, Tle, Ala(t-Bu), or Cha
DCTYHXGELVWCT

SEQ ID NO: 47 - protein, 13 aa, synthetic construct
  REGION 1..13: note = IgG binding peptide
  SITE 6: note = MISC_FEATURE - X is K, C, D, E, R, V, F, L, 2-Aminooctanedioic acid, Dpr, Orn,AcOrn, AcDab, Dab, Nle, Nva, Tle, Ala(t-Bu), or Cha
DCAWHXGELVWCT

SEQ ID NO: 48 - protein, 13 aa, synthetic construct
  REGION 1..13: note = IgG binding peptide
  SITE 6: note = MISC_FEATURE - X is K, C, D, E, R, V, F, L, 2-Aminooctanedioic acid, Dpr, Orn,AcOrn, AcDab, Dab, Nle, Nva, Tle, Ala(t-Bu), or Cha
DCTYTXGNLVWCT

SEQ ID NO: 49 - protein, 13 aa, synthetic construct
  REGION 1..13: note = IgG binding peptide
  SITE 6: note = MISC_FEATURE - X is K, C, D, E, R, V, F, L, 2-Aminooctanedioic acid, Dpr, Orn,AcOrn, AcDab, Dab, Nle, Nva, Tle, Ala(t-Bu), or Cha
DCAYTXGNLVWCT

SEQ ID NO: 50 - protein, 13 aa, synthetic construct
  REGION 1..13: note = IgG binding peptide
  SITE 6: note = MISC_FEATURE - X is K, C, D, E, R, V, F, L, 2-Aminooctanedioic acid, Dpr, Orn,AcOrn, AcDab, Dab, Nle, Nva, Tle, Ala(t-Bu), or Cha
DCSYTXGNLVWCT

SEQ ID NO: 51 - protein, 13 aa, synthetic construct
  REGION 1..13: note = IgG binding peptide
  SITE 6: note = MISC_FEATURE - X is K, C, D, E, R, V, F, L, 2-Aminooctanedioic acid, Dpr, Orn,AcOrn, AcDab, Dab, Nle, Nva, Tle, Ala(t-Bu), or Cha
DCTWTXGNLVWCT

SEQ ID NO: 52 - protein, 13 aa, synthetic construct
  REGION 1..13: note = IgG binding peptide
  SITE 6: note = MISC_FEATURE - X is K, C, D, E, R, V, F, L, 2-Aminooctanedioic acid, Dpr, Orn,AcOrn, AcDab, Dab, Nle, Nva, Tle, Ala(t-Bu), or Cha
DCTYHXGNLVWCT

SEQ ID NO: 53 - protein, 13 aa, synthetic construct
  REGION 1..13: note = IgG binding peptide
  SITE 6: note = MISC_FEATURE - X is K, C, D, E, R, V, F, L, 2-Aminooctanedioic acid, Dpr, Orn,AcOrn, AcDab, Dab, Nle, Nva, Tle, Ala(t-Bu), or Cha
DCTYRXGNLVWCT

SEQ ID NO: 54 - protein, 13 aa, synthetic construct
  REGION 1..13: note = IgG binding peptide
  SITE 6: note = MISC_FEATURE - X is K, C, D, E, R, V, F, L, 2-Aminooctanedioic acid, Dpr, Orn,AcOrn, AcDab, Dab, Nle, Nva, Tle, Ala(t-Bu), or Cha
DCTYSXGNLVWCT

SEQ ID NO: 55 - protein, 13 aa, synthetic construct
  REGION 1..13: note = IgG binding peptide
  SITE 6: note = MISC_FEATURE - X is K, C, D, E, R, V, F, L, 2-Aminooctanedioic acid, Dpr, Orn,AcOrn, AcDab, Dab, Nle, Nva, Tle, Ala(t-Bu), or Cha
DCTYTXGNLVWCT

SEQ ID NO: 56 - protein, 13 aa, synthetic construct
  REGION 1..13: note = IgG binding peptide
  SITE 6: note = MISC_FEATURE - X is K, C, D, E, R, V, F, L, 2-Aminooctanedioic acid, Dpr, Orn,AcOrn, AcDab, Dab, Nle, Nva, Tle, Ala(t-Bu), or Cha
DCTYTXGELVWCT

SEQ ID NO: 57 - protein, 13 aa, synthetic construct
  REGION 1..13: note = IgG binding peptide
  SITE 6: note = MISC_FEATURE - X is K, C, D, E, R, V, F, L, 2-Aminooctanedioic acid, Dpr, Orn,AcOrn, AcDab, Dab, Nle, Nva, Tle, Ala(t-Bu), or Cha
DCTYTXGRLVWCT

SEQ ID NO: 58 - protein, 13 aa, synthetic construct
  REGION 1..13: note = IgG binding peptide
  SITE 6: note = MISC_FEATURE - X is K, C, D, E, R, V, F, L, 2-Aminooctanedioic acid, Dpr, Orn,AcOrn, AcDab, Dab, Nle, Nva, Tle, Ala(t-Bu), or Cha
DCTYTXGDLVWCT

SEQ ID NO: 59 - protein, 13 aa, synthetic construct
  REGION 1..13: note = IgG binding peptide
  SITE 6: note = MISC_FEATURE - X is K, C, D, E, R, V, F, L, 2-Aminooctanedioic acid, Dpr, Orn,AcOrn, AcDab, Dab, Nle, Nva, Tle, Ala(t-Bu), or Cha
DCTYTXGNLIWCT

SEQ ID NO: 60 - protein, 13 aa, synthetic construct
  REGION 1..13: note = IgG binding peptide
DCAYHRGELVWCT

SEQ ID NO: 61 - protein, 17 aa, synthetic construct
  REGION 1..17: note = IgG binding peptide
GPDCAYHRGELVWCTFH

SEQ ID NO: 62 - protein, 13 aa, synthetic construct
  REGION 1..13: note = IgG binding peptide
RCAYHRGELVWCS

SEQ ID NO: 63 - protein, 17 aa, synthetic construct
  REGION 1..17: note = IgG binding peptide
GPRCAYHRGELVWCSFH

SEQ ID NO: 64 - protein, 17 aa, synthetic construct
  REGION 1..17: note = IgG binding peptide
SPDCAYHRGELVWCTFH

SEQ ID NO: 65 - protein, 17 aa, synthetic construct
  REGION 1..17: note = IgG binding peptide
GDDCAYHRGELVWCTFH

SEQ ID NO: 66 - protein, 17 aa, synthetic construct
  REGION 1..17: note = IgG binding peptide
GPSCAYHRGELVWCTFH

SEQ ID NO: 67 - protein, 17 aa, synthetic construct
  REGION 1..17: note = IgG binding peptide
GPDCAYHRGELVWCSFH

SEQ ID NO: 68 - protein, 17 aa, synthetic construct
  REGION 1..17: note = IgG binding peptide
GPDCAYHRGELVWCTHH

SEQ ID NO: 69 - protein, 17 aa, synthetic construct
  REGION 1..17: note = IgG binding peptide
GPDCAYHRGELVWCTFY

SEQ ID NO: 70 - protein, 17 aa, synthetic construct
  REGION 1..17: note = IgG binding peptide
SPDCAYHRGELVWCTFY

SEQ ID NO: 71 - protein, 17 aa, synthetic construct
  REGION 1..17: note = IgG binding peptide
SDDCAYHRGELVWCTFY

SEQ ID NO: 72 - protein, 13 aa, synthetic construct
  REGION 1..13: note = IgG binding peptide
DCTYHRGNLVWCT

SEQ ID NO: 73 - protein, 13 aa, synthetic construct
  REGION 1..13: note = IgG binding peptide
DCAYHRGNLVWCT

SEQ ID NO: 74 - protein, 13 aa, synthetic construct
  REGION 1..13: note = IgG binding peptide
DCTYHRGELVWCT

SEQ ID NO: 75 - protein, 13 aa, synthetic construct
  REGION 1..13: note = IgG binding peptide
DCAWHRGELVWCT

SEQ ID NO: 76 - protein, 13 aa, synthetic construct
  REGION 1..13: note = IgG binding peptide
DCTYTNGNLVWCT

SEQ ID NO: 77 - protein, 13 aa, synthetic construct
  REGION 1..13: note = IgG binding peptide
DCAYTNGNLVWCT

SEQ ID NO: 78 - protein, 13 aa, synthetic construct
  REGION 1..13: note = IgG binding peptide
DCSYTNGNLVWCT

SEQ ID NO: 79 - protein, 13 aa, synthetic construct
  REGION 1..13: note = IgG binding peptide
DCTWTNGNLVWCT

SEQ ID NO: 80 - protein, 13 aa, synthetic construct
  REGION 1..13: note = IgG binding peptide
DCTYHNGNLVWCT

SEQ ID NO: 81 - protein, 13 aa, synthetic construct
  REGION 1..13: note = IgG binding peptide
DCTYRNGNLVWCT

SEQ ID NO: 82 - protein, 13 aa, synthetic construct
  REGION 1..13: note = IgG binding peptide
DCTYSNGNLVWCT

SEQ ID NO: 83 - protein, 13 aa, synthetic construct
  REGION 1..13: note = IgG binding peptide
DCTYTRGNLVWCT

SEQ ID NO: 84 - protein, 13 aa, synthetic construct
  REGION 1..13: note = IgG binding peptide
DCTYTNGELVWCT

SEQ ID NO: 85 - protein, 13 aa, synthetic construct
  REGION 1..13: note = IgG binding peptide
DCTYTNGRLVWCT

SEQ ID NO: 86 - protein, 13 aa, synthetic construct
  REGION 1..13: note = IgG binding peptide
DCTYTNGDLVWCT

SEQ ID NO: 87 - protein, 13 aa, synthetic construct
  REGION 1..13: note = IgG binding peptide
DCTYTNGNLIWCT

SEQ ID NO: 88 - protein, 22 aa, synthetic construct
  REGION 1..22: note = IgG binding peptide
GSGGSGPDCAYHRGELVWCTFH

SEQ ID NO: 89 - protein, 18 aa, synthetic construct
  REGION 1..18: note = IgG binding peptide
GSGGSDCAYHRGELVWCT

SEQ ID NO: 90 - protein, 23 aa, synthetic construct
  REGION 1..23: note = IgG binding peptide
KRRRGSGPDCAYHKGELVWCTFH

SEQ ID NO: 91 - protein, 23 aa, synthetic construct
  REGION 1..23: note = IgG binding peptide
KEEGGSGPDCAYHKGELVWCTFH

SEQ ID NO: 92 - protein, 17 aa, synthetic construct
  REGION 1..17: note = IgG binding peptide
GPDCAYHKGELVWCTFH

SEQ ID NO: 93 - protein, 22 aa, synthetic construct
  REGION 1..22: note = IgG binding peptide
RRRGSGPDCAYHKGELVWCTFH

SEQ ID NO: 94 - protein, 22 aa, synthetic construct
  REGION 1..22: note = IgG binding peptide
EEGGSGPDCAYHKGELVWCTFH

SEQ ID NO: 95 - protein, 19 aa, synthetic construct
  REGION 1..19: note = IgG binding peptide
KRRRGSDCAYHKGELVWCT

SEQ ID NO: 96 - protein, 19 aa, synthetic construct
  REGION 1..19: note = IgG binding peptide
KEEGGSDCAYHKGELVWCT

SEQ ID NO: 97 - protein, 13 aa, synthetic construct
  REGION 1..13: note = IgG binding peptide
DCAYHKGELVWCT

SEQ ID NO: 98 - protein, 18 aa, synthetic construct
  REGION 1..18: note = IgG binding peptide
RRRGSDCAYHKGELVWCT

SEQ ID NO: 99 - protein, 18 aa, synthetic construct
  REGION 1..18: note = IgG binding peptide
EEGGSDCAYHKGELVWCT

SEQ ID NO: 100 - protein, 34 aa, synthetic construct
  REGION 1..34: note = IgG binding peptide
FNMQCQRRFYEALHDPNLNEEQRNARIRSIRDDC

SEQ ID NO: 101 - protein, 35 aa, synthetic construct
  REGION 1..35: note = IgG binding peptide
GFNMQCQRRFYEALHDPNLNEEQRNARIRSIRDDC

SEQ ID NO: 102 - protein, 34 aa, synthetic construct
  REGION 1..34: note = IgG binding peptide
KNMQCQRRFYEALHDPNLNEEQRNARIRSIRDDC

SEQ ID NO: 103 - protein, 35 aa, synthetic construct
  REGION 1..35: note = IgG binding peptide
GFNMQCQKRFYEALHDPNLNEEQRNARIRSIRDDC

SEQ ID NO: 104 - protein, 34 aa, synthetic construct
  REGION 1..34: note = IgG binding peptide
KNMQCQKRFYEALHDPNLNEEQRNARIRSIRDDC

SEQ ID NO: 105 - protein, 33 aa, synthetic construct
  REGION 1..33: note = IgG binding peptide
FNMQQQRRFYEALHDPNLNEEQRNARIRSIRDD

SEQ ID NO: 106 - protein, 35 aa, synthetic construct
  REGION 1..35: note = IgG binding peptide
GKNMQCQRRFYEALHDPNLNEEQRNARIRSIRDDC

SEQ ID NO: 107 - protein, 40 aa, synthetic construct
  REGION 1..40: note = IgG binding peptide
FNMQQQRRFYEALHDPNLNEEQRNARIRSIRDDPSGSGSK

SEQ ID NO: 108 - protein, 40 aa, synthetic construct
  REGION 1..40: note = IgG binding peptide
FNMQCQRRFYEALHDPNLNEEQRNARIRSIRDDCSGSGSK

SEQ ID NO: 109 - protein, 34 aa, synthetic construct
  REGION 1..34: note = IgG binding peptide
FNMQQQRRFYEALHDPNLNEEQRNARIRSIRDDP

SEQ ID NO: 110 - protein, 33 aa, synthetic construct
  REGION 1..33: note = IgG binding peptide
FNMQQQCRFYEALHDPNLNEEQRNARIRSIRDD

SEQ ID NO: 111 - protein, 34 aa, synthetic construct
  REGION 1..34: note = IgG binding peptide
FNMQQQRRFYEALHDPNLNEEQRNARIRSIRDDC

SEQ ID NO: 112 - protein, 39 aa, synthetic construct
  REGION 1..39: note = IgG binding peptide
FNMQQQRRFYEALHDPNLNEEQRNARIRSIRDDPSRRKR

SEQ ID NO: 113 - protein, 39 aa, synthetic construct
  REGION 1..39: note = IgG binding peptide
FNMQQQRRFYEALHDPNLNEEQRNARIRSIRDDPSRRCR

SEQ ID NO: 114 - protein, 44 aa, synthetic construct
  REGION 1..44: note = IgG binding peptide
FNMQQQCRFYEALHDPNLNEEQRNARICSIRDDPSRRCRRCRRC

SEQ ID NO: 115 - protein, 44 aa, synthetic construct
  REGION 1..44: note = IgG binding peptide
FNMQQQKRFYEALHDPNLNEEQRNARIKSIRDDPSRRKRRKRRK

SEQ ID NO: 116 - protein, 33 aa, synthetic construct
  REGION 1..33: note = IgG binding peptide
KNMQQQCRFYEALHDPNLNEEQRNARIRSIRDD

SEQ ID NO: 117 - protein, 34 aa, synthetic construct
  REGION 1..34: note = IgG binding peptide
KNMQQQRRFYEALHDPNLNEEQRNARIRSIRDDC

SEQ ID NO: 118 - protein, 39 aa, synthetic construct
  REGION 1..39: note = IgG binding peptide
KNMQQQRRFYEALHDPNLNEEQRNARIRSIRDDPSRRKR

SEQ ID NO: 119 - protein, 39 aa, synthetic construct
  REGION 1..39: note = IgG binding peptide
KNMQQQRRFYEALHDPNLNEEQRNARIRSIRDDPSRRCR

SEQ ID NO: 120 - protein, 44 aa, synthetic construct
  REGION 1..44: note = IgG binding peptide
KNMQQQCRFYEALHDPNLNEEQRNARICSIRDDPSRRCRRCRRC

SEQ ID NO: 121 - protein, 44 aa, synthetic construct
  REGION 1..44: note = IgG binding peptide
KNMQQQKRFYEALHDPNLNEEQRNARIKSIRDDPSRRKRRKRRK

SEQ ID NO: 122 - protein, 34 aa, synthetic construct
  REGION 1..34: note = IgG binding peptide
GFNMQQQCRFYEALHDPNLNEEQRNARIRSIRDD

SEQ ID NO: 123 - protein, 35 aa, synthetic construct
  REGION 1..35: note = IgG binding peptide
GFNMQQQRRFYEALHDPNLNEEQRNARIRSIRDDC

SEQ ID NO: 124 - protein, 40 aa, synthetic construct
  REGION 1..40: note = IgG binding peptide
GFNMQQQRRFYEALHDPNLNEEQRNARIRSIRDDPSRRKR

SEQ ID NO: 125 - protein, 40 aa, synthetic construct
  REGION 1..40: note = IgG binding peptide
GFNMQQQRRFYEALHDPNLNEEQRNARIRSIRDDPSRRCR

SEQ ID NO: 126 - protein, 45 aa, synthetic construct
  REGION 1..45: note = IgG binding peptide
GFNMQQQCRFYEALHDPNLNEEQRNARICSIRDDPSRRCRRCRRC

SEQ ID NO: 127 - protein, 45 aa, synthetic construct
  REGION 1..45: note = IgG binding peptide
GFNMQQQKRFYEALHDPNLNEEQRNARIKSIRDDPSRRKRRKRRK

SEQ ID NO: 128 - protein, 34 aa, synthetic construct
  REGION 1..34: note = IgG binding peptide
FNMQCQZRFYEALHDPNLNEEQRNARIRSIRDDC

SEQ ID NO: 129 - protein, 34 aa, synthetic construct
  REGION 1..34: note = IgG binding peptide
KNMQCQZRFYEALHDPNLNEEQRNARIRSIRDDC

SEQ ID NO: 130 - protein, 40 aa, synthetic construct
  REGION 1..40: note = IgG binding peptide
GFNMQCQKRFYEALHDPNLNEEQRNARIRSIRDDCSRRKR

SEQ ID NO: 131 - protein, 34 aa, synthetic construct
  REGION 1..34: note = IgG binding peptide
FNMQCQKRFYEALHDPNLNEEQRNARIRSIRDDC

SEQ ID NO: 132 - protein, 39 aa, synthetic construct
  REGION 1..39: note = IgG binding peptide
KNMQCQKRFYEALHDPNLNEEQRNARIRSIRDDCSRRKR

SEQ ID NO: 133 - protein, 45 aa, synthetic construct
  REGION 1..45: note = IgG binding peptide
GFNMQCQKRFYEALHDPNLNEEQRNARIRSIRDDCSRRKRRKRRK

SEQ ID NO: 134 - protein, 44 aa, synthetic construct
  REGION 1..44: note = IgG binding peptide
KNMQCQKRFYEALHDPNLNEEQRNARIRSIRDDCSRRKRRKRRK

SEQ ID NO: 135 - protein, 45 aa, synthetic construct; identical to SEQ ID NO: 133
  REGION 1..45: note = IgG binding peptide

SEQ ID NO: 136 - protein, 11 aa, synthetic construct
  REGION 1..11: note = IgG binding peptide
CAWHLGELVWC

SEQ ID NO: 137 - protein, 13 aa, synthetic construct
  REGION 1..13: note = IgG binding peptide
DCAWHLGELVWCT

SEQ ID NO: 138 - protein, 13 aa, synthetic construct
  REGION 1..13: note = IgG binding peptide
DCAWHLGELVFCT

SEQ ID NO: 139 - protein, 13 aa, synthetic construct
  REGION 1..13: note = IgG binding peptide
  SITE 11: note = MISC_FEATURE - X is 1-naphtoyl, 2-naphtoyl, benzyl, or benzothiophene
DCAWHLGELVXCT

SEQ ID NO: 140 - protein, 15 aa, synthetic construct
  REGION 1..15: note = IgG binding peptide
CDCAWHLGELVWCTC

SEQ ID NO: 141 - protein, 11 aa, synthetic construct
  REGION 1..11: note = IgG binding peptide
CAYHLGELVWC

SEQ ID NO: 142 - protein, 14 aa, synthetic construct
  REGION 1..14: note = IgG binding peptide
DCAYHLGELVWCTF

SEQ ID NO: 143 - protein, 23 aa, synthetic construct
  REGION 1..23: note = IgG binding peptide
KRRRGSGPDCAYHKGELVWCTFH

SEQ ID NO: 144 - protein, 33 aa, synthetic construct
  REGION 1..33: note = IgG binding peptide
NMQCQRRFYEALHDPNLNEEQRNARIRSIRDDC

SEQ ID NO: 145 - protein, 34 aa, synthetic construct; identical to SEQ ID NO: 100
  REGION 1..34: note = IgG binding peptide

SEQ ID NO: 146 - protein, 33 aa, synthetic construct; identical to SEQ ID NO: 144
  REGION 1..33: note = IgG binding peptide

SEQ ID NO: 147 - protein, 34 aa, synthetic construct; identical to SEQ ID NO: 131
  REGION 1..34: note = IgG binding peptide

SEQ ID NO: 148 - protein, 33 aa, synthetic construct
  REGION 1..33: note = IgG binding peptide
NMQCQKRFYEALHDPNLNEEQRNARIRSIRDDC

SEQ ID NO: 149 - protein, 32 aa, synthetic construct
  REGION 1..32: note = IgG binding peptide
NMQQQRRFYEALHDPNLNEEQRNARIRSIRDD

SEQ ID NO: 150 - protein, 34 aa, synthetic construct; identical to SEQ ID NO: 102
  REGION 1..34: note = IgG binding peptide

SEQ ID NO: 151 - protein, 39 aa, synthetic construct
  REGION 1..39: note = IgG binding peptide
NMQQQRRFYEALHDPNLNEEQRNARIRSIRDDPSGSGSK

SEQ ID NO: 152 - protein, 39 aa, synthetic construct
  REGION 1..39: note = IgG binding peptide
NMQCQRRFYEALHDPNLNEEQRNARIRSIRDDCSGSGSK

SEQ ID NO: 153 - protein, 33 aa, synthetic construct
  REGION 1..33: note = IgG binding peptide
NMQQQRRFYEALHDPNLNEEQRNARIRSIRDDP

SEQ ID NO: 154 - protein, 32 aa, synthetic construct
  REGION 1..32: note = IgG binding peptide
NMQQQCRFYEALHDPNLNEEQRNARIRSIRDD

SEQ ID NO: 155 - protein, 33 aa, synthetic construct
  REGION 1..33: note = IgG binding peptide
NMQQQRRFYEALHDPNLNEEQRNARIRSIRDDC

SEQ ID NO: 156 - protein, 38 aa, synthetic construct
  REGION 1..38: note = IgG binding peptide
NMQQQRRFYEALHDPNLNEEQRNARIRSIRDDPSRRKR

SEQ ID NO: 157 - protein, 38 aa, synthetic construct
  REGION 1..38: note = IgG binding peptide
NMQQQRRFYEALHDPNLNEEQRNARIRSIRDDPSRRCR

SEQ ID NO: 158 - protein, 43 aa, synthetic construct
  REGION 1..43: note = IgG binding peptide
NMQQQCRFYEALHDPNLNEEQRNARICSIRDDPSRRCRRCRRC

SEQ ID NO: 159 - protein, 43 aa, synthetic construct
  REGION 1..43: note = IgG binding peptide
NMQQQKRFYEALHDPNLNEEQRNARIKSIRDDPSRRKRRKRRK

SEQ ID NO: 160 - protein, 32 aa, synthetic construct; identical to SEQ ID NO: 154
  REGION 1..32: note = IgG binding peptide

SEQ ID NO: 161 - protein, 33 aa, synthetic construct; identical to SEQ ID NO: 155
  REGION 1..33: note = IgG binding peptide

SEQ ID NO: 162 - protein, 38 aa, synthetic construct; identical to SEQ ID NO: 156
  REGION 1..38: note = IgG binding peptide

SEQ ID NO: 163 - protein, 38 aa, synthetic construct; identical to SEQ ID NO: 157
  REGION 1..38: note = IgG binding peptide

SEQ ID NO: 164 - protein, 43 aa, synthetic construct; identical to SEQ ID NO: 158
  REGION 1..43: note = IgG binding peptide

SEQ ID NO: 165 - protein, 43 aa, synthetic construct; identical to SEQ ID NO: 159
  REGION 1..43: note = IgG binding peptide

SEQ ID NO: 166 - protein, 33 aa, synthetic construct; identical to SEQ ID NO: 110
  REGION 1..33: note = IgG binding peptide

SEQ ID NO: 167 - protein, 34 aa, synthetic construct; identical to SEQ ID NO: 111
  REGION 1..34: note = IgG binding peptide

SEQ ID NO: 168 - protein, 39 aa, synthetic construct; identical to SEQ ID NO: 112
  REGION 1..39: note = IgG binding peptide

SEQ ID NO: 169 - protein, 39 aa, synthetic construct; identical to SEQ ID NO: 113
  REGION 1..39: note = IgG binding peptide

SEQ ID NO: 170 - protein, 44 aa, synthetic construct; identical to SEQ ID NO: 114
  REGION 1..44: note = IgG binding peptide

SEQ ID NO: 171 - protein, 44 aa, synthetic construct; identical to SEQ ID NO: 115
  REGION 1..44: note = IgG binding peptide

SEQ ID NO: 172 - protein, 33 aa, synthetic construct
  REGION 1..33: note = IgG binding peptide
NMQCQZRFYEALHDPNLNEEQRNARIRSIRDDC

SEQ ID NO: 173 - protein, 33 aa, synthetic construct; identical to SEQ ID NO: 172
  REGION 1..33: note = IgG binding peptide

SEQ ID NO: 174 - protein, 39 aa, synthetic construct
  REGION 1..39: note = IgG binding peptide
FNMQCQKRFYEALHDPNLNEEQRNARIRSIRDDCSRRKR

SEQ ID NO: 175 - protein, 33 aa, synthetic construct; identical to SEQ ID NO: 148
  REGION 1..33: note = IgG binding peptide

SEQ ID NO: 176 - protein, 38 aa, synthetic construct
  REGION 1..38: note = IgG binding peptide
NMQCQKRFYEALHDPNLNEEQRNARIRSIRDDCSRRKR

SEQ ID NO: 177 - protein, 44 aa, synthetic construct
  REGION 1..44: note = IgG binding peptide
FNMQCQKRFYEALHDPNLNEEQRNARIRSIRDDCSRRKRRKRRK

SEQ ID NO: 178 - protein, 43 aa, synthetic construct
  REGION 1..43: note = IgG binding peptide
NMQCQKRFYEALHDPNLNEEQRNARIRSIRDDCSRRKRRKRRK

SEQ ID NO: 179 - protein, 44 aa, synthetic construct; identical to SEQ ID NO: 177
  REGION 1..44: note = IgG binding peptide

SEQ ID NO: 180 - protein, 8 aa, synthetic construct
  source 1..8: note = GPA33-2RmhC-2 VH CDR1
GYTFTGYY

SEQ ID NO: 181 - protein, 8 aa, synthetic construct
  source 1..8: note = VH CDR1
GFTFSTYN

SEQ ID NO: 182 - protein, 8 aa, synthetic construct
  source 1..8: note = GPA33-2RmhC-11 VH CDR1
GFTFSSYA

SEQ ID NO: 183 - protein, 8 aa, synthetic construct
  source 1..8: note = VH CDR1
GGTFSSYA

SEQ ID NO: 184 - protein, 8 aa, synthetic construct
  source 1..8: note = VH CDR1
GFTFDDYA

SEQ ID NO: 185 - protein, 8 aa, synthetic construct
  source 1..8: note = GPA33-2RmhC-23 VH CDR1
GFTFGDYG

SEQ ID NO: 186 - protein, 8 aa, synthetic construct
  source 1..8: note = GPA33-2RmhC-28 VH CDR1
GYTFTNYG

SEQ ID NO: 187 - protein, 10 aa, synthetic construct
  source 1..10: note = GPA33-2RmhC-29 VH CDR1
GGSVSSTSYY

SEQ ID NO: 188 - protein, 8 aa, synthetic construct
  source 1..8: note = GPA33-2RmhC-36 VH CDR1
GFTFSNFN

SEQ ID NO: 189 - protein, 8 aa, synthetic construct
  source 1..8: note = GPA33-2RmhC-37 VH CDR1
GGSISSYY

SEQ ID NO: 190 - protein, 8 aa, synthetic construct
  source 1..8: note = GPA33-2RmhC-40 VH CDR1
GFTFSNYA

SEQ ID NO: 191 - protein, 8 aa, synthetic construct
  source 1..8: note = GPA33-2RmhC-44 VH CDR1
GYTLTELS

SEQ ID NO: 192 - protein, 10 aa, synthetic construct
  source 1..10: note = GPA33-2RmhC-45 VH CDR1
GGSVTSTSYY

SEQ ID NO: 193 - protein, 10 aa, synthetic construct
  source 1..10: note = GPA33-2RmhC-47
GDSVSSNSAA

SEQ ID NO: 194 - protein, 8 aa, synthetic construct
  source 1..8: note = GPA33-2RmhC-48 VH CDR1
GGTFNTYA

SEQ ID NO: 195 - protein, 8 aa, synthetic construct
  source 1..8: note = GPA33-2RmhC-49 VH CDR1
GFTFSSYG

SEQ ID NO: 196 - protein, 8 aa, synthetic construct
  source 1..8: note = GPA33-2RmhC-50 VH CDR1
GYSFTDSW

SEQ ID NO: 197 - protein, 8 aa, synthetic construct
  source 1..8: note = VH CDR2
ISSRGDYI

SEQ ID NO: 198 - protein, 8 aa, synthetic construct
  source 1..8: note = GPA33-2RmhC-2 VH CDR2
INPNSGGT

SEQ ID NO: 199 - protein, 8 aa, synthetic construct
  source 1..8: note = VH CDR2
IDRSSTYI

SEQ ID NO: 200 - protein, 8 aa, synthetic construct
  source 1..8: note = VH CDR2
ISSSGDYI

SEQ ID NO: 201 - protein, 8 aa, synthetic construct
  source 1..8: note = GPA33-2RmhC-8 VH CDR2
IVSSGDYI

SEQ ID NO: 202 - protein, 8 aa, synthetic construct
  source 1..8: note = VH CDR2
ISGSGGST

SEQ ID NO: 203 - protein, 8 aa, synthetic construct
  source 1..8: note = VH CDR2
IIPIFGTA

SEQ ID NO: 204 - protein, 8 aa, synthetic construct
  source 1..8: note = VH CDR2
ISRDSAYI

SEQ ID NO: 205 - protein, 8 aa, synthetic construct
  source 1..8: note = VH CDR2
ISWNSGSI

SEQ ID NO: 206 - protein, 8 aa, synthetic construct
  source 1..8: note = GPA33-2RmhC-23 VH CDR2
ISWNSGRK

SEQ ID NO: 207 - protein, 8 aa, synthetic construct
  source 1..8: note = GPA33-2RmhC-28 VH CDR2
ISAYNGNT

SEQ ID NO: 208 - protein, 7 aa, synthetic construct
  source 1..7: note = VH CDR2
IYYSGST

SEQ ID NO: 209 - protein, 8 aa, synthetic construct
  source 1..8: note = GPA33-2RmhC-32 VH CDR2
ISWSSGSI

SEQ ID NO: 210 - protein, 7 aa, synthetic construct
  source 1..7: note = GPA33-2RmhC-37 VH CDR2
IYHSGST

SEQ ID NO: 211 - protein, 8 aa, synthetic construct
  source 1..8: note = GPA33-2RmhC-39 VH CDR2
ISSSGDYM

SEQ ID NO: 212 - protein, 8 aa, synthetic construct
  source 1..8: note = GPA33-2RmhC-44
FDPEDGET

SEQ ID NO: 213 - protein, 9 aa, synthetic construct
  source 1..9: note = GPA33-2RmhC-47 VH CDR2
TYYRSKWYN

SEQ ID NO: 214 - protein, 8 aa, synthetic construct
  source 1..8: note = GPA33-2RmhC-48 VH CDR2
IIPIFGSA

SEQ ID NO: 215 - protein, 8 aa, synthetic construct
  source 1..8: note = GPA33-2RmhC-49 VH CDR2
ISTSSSSI

SEQ ID NO: 216 - protein, 8 aa, synthetic construct
  source 1..8: note = GPA33-2RmhC-50 VH CDR2
IYPGDSDT

SEQ ID NO: 217 - protein, 11 aa, synthetic construct
  source 1..11: note = VH CDR3
AREAVGTPFDY

SEQ ID NO: 218 - protein, 10 aa, synthetic construct
  source 1..10: note = GPA33-2RmhC-2 VH CDR3
ARVESGAFDI

SEQ ID NO: 219 - protein, 11 aa, synthetic construct
  source 1..11: note = VH CDR3
AREAIGTPFDY

SEQ ID NO: 220 - protein, 15 aa, synthetic construct
  source 1..15: note = GPA33-2RmhC-11 VH CDR3
AKGDIVVVPAALFDY

SEQ ID NO: 221 - protein, 17 aa, synthetic construct
  source 1..17: note = GPA33-2RmhC-14 VH CDR3
ARGQQQLAYYQFYGMDV

SEQ ID NO: 222 - protein, 11 aa, synthetic construct
  source 1..11: note = VH CDR3
VREGVAGAFDI

SEQ ID NO: 223 - protein, 11 aa, synthetic construct
  source 1..11: note = GPA33-2RmhC-19 VH CDR3
VREGVAGAFGI

SEQ ID NO: 224 - protein, 17 aa, synthetic construct
  source 1..17: note = GPA33-2RmhC-20 VH CDR3
ARAYGGSAYYYNYGMDV

SEQ ID NO: 225 - protein, 17 aa, synthetic construct
  source 1..17: note = GPA33-2RmhC-21 VH CDR3
AKDRWDTAMITPDAFDI

SEQ ID NO: 226 - protein, 17 aa, synthetic construct
  source 1..17: note = GPA33-2RmhC-23 VH CDR3
AKDMKIIRMEAAGPLEF

SEQ ID NO: 227 - protein, 17 aa, synthetic construct
  source 1..17: note = GPA33-2RmhC-27 VH CDR3
ARAYGGSAYYHNYGMDV

SEQ ID NO: 228 - protein, 15 aa, synthetic construct
  source 1..15: note = GPA33-2RmhC-28 VH CDR3
ARDSPLNWGPDAFDI

SEQ ID NO: 229 - protein, 15 aa, synthetic construct
  source 1..15: note = VH CDR3
ARDRGSGWYRDAFDI

SEQ ID NO: 230 - protein, 15 aa, synthetic construct
  source 1..15: note = GPA33-2RmhC-32 VH CDR3
AKDITDSSGYYGMDA

SEQ ID NO: 231 - protein, 11 aa, synthetic construct
  source 1..11: note = GPA33-2RmhC-35 VH CDR3
AREGPGTPLDY

SEQ ID NO: 232 - protein, 18 aa, synthetic construct
  source 1..18: note = GPA33-2RmhC-37 VH CDR3
ARSRQQLLRDYYYYGMDV

SEQ ID NO: 233 - protein, 19 aa, synthetic construct
  source 1..19: note = GPA33-2RmhC-40 VH CDR3
AKGSGSYYKPVYYYYGMDV

SEQ ID NO: 234 - protein, 14 aa, synthetic construct
  source 1..14: note = GPA33-2RmhC-42 VH CDR3
AKCDGSGSYGAFDI

SEQ ID NO: 235 - protein, 19 aa, synthetic construct
  source 1..19: note = GPA33-2RmhC-43 VH CDR3
ARAPDILTSSGYYYYGMDV

SEQ ID NO: 236 - protein, 13 aa, synthetic construct
  source 1..13: note = GPA33-2RmhC-44 VH CDR3
ATEAAAGTPFFDY

SEQ ID NO: 237 - protein, 14 aa, synthetic construct
  source 1..14: note = GPA33-2RmhC-46 VH CDR3
AKDIGAVAGYGMDV

SEQ ID NO: 238 - protein, 13 aa, synthetic construct
  source 1..13: note = GPA33-2RmhC-47 VH CDR3
AREKTGLYWYFDL

SEQ ID NO: 239 - protein, 17 aa, synthetic construct
  source 1..17: note = GPA33-2RmhC-48 VH CDR3
ARAYGGSAHYYSYGMDV

SEQ ID NO: 240 - protein, 19 aa, synthetic construct
  source 1..19: note = GPA33-2RmhC-49 VH CDR3
ARDGAYCGGDCYPYWNFDL

SEQ ID NO: 241 - protein, 11 aa, synthetic construct
  source 1..11: note = GPA33-2RmhC-50 VH CDR3
ARPYRDYSFDY

SEQ ID NO: 242 - protein, 118 aa, synthetic construct
  source 1..118: note = GPA33-2RmhC-1 VH
QVQLQESGGGLVKPGGSLRLSCAASGFTFSSYNMNWVRQAPGKGLEWVSSISSRGDYIYYADSVKGRFTISRDNAKNSLYLQMSSLRAEDTAVYYCAREAVGTPFDYWGQGTLVTVSS

SEQ ID NO: 243 - protein, 117 aa, synthetic construct
  source 1..117: note = GPA33-2RmhC-2 VH
QMQLVQSGAEVKKPGASVKVSCKASGYTFTGYYMHWVRQAPGRGLEWMGRINPNSGGTNYAQKFQGRVTMTRDTSISTAYMELSRLRSDDTVVYYCARVESGAFDIWGQGTMVTVSS

SEQ ID NO: 244 - protein, 118 aa, synthetic construct
  source 1..118: note = GPA33-2RmhC-3 VH
QVQLVQSGGGLVKPGGSLRLSCAASGFTFSNYNMNWVRQAPGKGLEWVSSIDRSSTYIYYADSVKGRFTISRDNAKNSLYLQMNSLRAEDTAVYYCAREAVGTPFDYWGQGTLVTVSS

SEQ ID NO: 245 - protein, 118 aa, synthetic construct
  source 1..118: note = GPA33-2RmhC-4 VH
QVQLVQSGGGLVKPGGSLRLSCAASGFTFSNYNMNWVRQAPGKGLEWVSSISSSGDYIYYADSVKGRFTISRDDAKNSLYLQMNSLRAEDTAVYYCAREAIGTPFDYWGQGTLVTVSS

SEQ ID NO: 246 - protein, 118 aa, synthetic construct
  source 1..118: note = GPA33-2RmhC-5 VH
EVQLVESGGGLVKPGGSLRLSCAASGFTFSTYNMNWVRQAPGKGLEWVSSISSSGDYIYYADSVKGRFTISRDDAKNSLYLQMNSLRAEDTAVYYCAREAIGTPFDYWGQGTLVTVSS

SEQ ID NO: 247 - protein, 118 aa, synthetic construct
  source 1..118: note = GPA33-2RmhC-6 VH
QVQLVESGGGLVKPGGSLRLSCAASGFTFSSYNMNWVRQAPGKGLEWVSSISSRGDYIYYADSVKGRFIISRDNAKNSLYLQMSSLRAEDTAVYYCAREAVGTPFDYWGQGTLVTVSS

SEQ ID NO: 248 - protein, 118 aa, synthetic construct
  source 1..118: note = GPA33-2RmhC-7 VH
QVQLVQSGGGLVKPGGSLRLSCAASGFTFSSYNMNWVRQAPGKGLEWVSSIDRSSTYIYYADSVKGRFTISRDNAKNSLYLQMNSLRAEDTAVYYCAREGPGTPFDYWGQGTLVTVSS

SEQ ID NO: 249 - protein, 118 aa, synthetic construct
  source 1..118: note = GPA33-2RmhC-8 VH
EVQLVESGGGLVKPGGSLRLSCAASGFTFSNYNMNWVRQAPGKGLEWVSSIVSSGDYIYYADSVKGRFTTSRDNAKNSLYLQMSSLRAEDTAVYYCAREAVGTPFDYWGQGTLVTVSS

SEQ ID NO: 250 - protein, 118 aa, synthetic construct
  source 1..118: note = GPA33-2RmhC-9 VH
QVQLVQSGGGLVKPGGSLRLSCAASGFTFSSYNMNWVRQAPGKGLEWVSSIDRSSTYIYYADSVKGRFTISRDNAKNSLYLQMNSLRAEDTAVYYCAREAVGTPFDYWGQGTLVTVSS

SEQ ID NO: 251 - protein, 118 aa, synthetic construct
  source 1..118: note = GPA33-2RmhC-10 VH
QVQLVQSGGGLVKPGGSLRLSCAASGFTFSTYNMNWVRQAPGKGLEWVSSISSSGDYIYYADSVKGRFTISRDDAKNSLYLQMNSLRAEDTAVYYCAREGPGTPFDYWGQGTLVTVSS

SEQ ID NO: 252 - protein, 122 aa, synthetic construct
  source 1..122: note = GPA33-2RmhC-11 VH
QVQLVESGGGLVQPGGSLRLSCAASGFTFSSYAMSWVRQAPGKGLEWVSAISGSGGSTYYADSVKGRFTISRDDSKNTLYLQMNSLRAEDTAVYYCAKGDIVVVPAALFDYWGQGTLVTVSS

SEQ ID NO: 253 - protein, 118 aa, synthetic construct
  source 1..118: note = GPA33-2RmhC-12 VH
QVQLVQSGGGLVKPGGSLRLSCAASGFTFSTYNMNWVRQAPGKGLEWVSSISSSGDYIYYADSVKGRFTISRDDAKNSLYLQMNSLRAEDTAVYYCAREAIGTPFDYWGQGTLVTVSS

SEQ ID NO: 254 - protein, 118 aa, synthetic construct
  source 1..118: note = GPA33-2RmhC-13 VH
QMQLVQSRGGLVKPGGSLRLSCAASGFTFSSYNMNWVRQAPGKGLEWVSSISSRGDYIYYADSVKGRFTISRDNAKNSLYLQMSSLRAEDTAVYYCAREAVGTPFDYWGQGTLVTVSS

SEQ ID NO: 255 - protein, 124 aa, synthetic construct
  source 1..124: note = GPA33-2RmhC-14 VH
QVQLVQSGAEVKKPGSSVKVSCKASGGTFSSYAINWVRQAPGQGLEWMGGIIPIFGTADYAQKFRGRVTITADESTSTAYMELSSLRSEDTAVYYCARGQQQLAYYQFYGMDVWGQGTTVTVSS

SEQ ID NO: 256 - protein, 118 aa, synthetic construct
  source 1..118: note = GPA33-2RmhC-15 VH
QMQLVQSEGGLVKPGGSLRLSCAASGFTFSSYNMNWVRQAPGKGLEWVSSISSSGDFMYYADSVKGRFTISRDNAKNSLYLQMSSLRAEDTAVYYCAREGPGTPFDYWGQGTLVTVSS

SEQ ID NO: 257 - protein, 118 aa, synthetic construct
  source 1..118: note = GPA33-2RmhC-16 VH
QVQLVQSGGGLVKPGGSLRLSCAASGFTFSNYNMNWVRQAPGKGLEWVSSISSSGDFMYYADSVKGRFTISRDDAKNSLYLQMNSLRAEDTAVYYCAREAIGTPFDYWGQGTLVTVSS

SEQ ID NO: 258 - protein, 118 aa, synthetic construct
  source 1..118: note = GPA33-2RmhC-17 VH
QVQLVQSGGGLVKPGGSLRLSCAASGFTFSTYSMNWVRQAPGKGLEWVSSISRDSAYIYYADSVKGRFTISRDNAKNSLYLQMNSLRAEDTAVYYCVREGVAGAFDIWGQGTMVTVSS

SEQ ID NO: 259 - protein, 118 aa, synthetic construct
  source 1..118: note = GPA33-2RmhC-18 VH
EVQLVESGGGLVKPGGSLRLSCAASGFTFSTYSMNWVRQAPGKGLEWVSSISRDSAYIYYADSVKGRFTISRDNAKNSLYLQMNSLRAEDTAVYYCVREGVAGAFDIWGQGTMVTVSS

SEQ ID NO: 260 - protein, 118 aa, synthetic construct
  source 1..118: note = GPA33-2RmhC-19 VH
QMQLVQSGGGLVKPGGSLRLSCAASGFTFSTYSMNWVRQAPGKGLEWVSSISRDSAYIYYADSVKDRFTISRDNAKNSLYLQMNSLRAEDTAVYYCVREGVAGAFGIWGQGTMVTASS

SEQ ID NO: 261 - protein, 124 aa, synthetic construct
  source 1..124: note = GPA33-2RmhC-20 VH
QVQLVQSGAEVKKPGSSVKVSCKASGGTFSSYAFNWVRQAPGQGLEWMGGIIPIFGTANYAQKFQGRVTITADESTSTAYMELSSLRSEDTAVYYCARAYGGSAYYYNYGMDVWGQGTTVTVSS

SEQ ID NO: 262 - protein, 124 aa, synthetic construct
  source 1..124: note = GPA33-2RmhC-21 VH
QVQLVESGGGLVQPGRSLRLSCAASGFTFDDYAMHWVRQAPGKGLEWVSGISWNSGSIGYADSVKGRFTISRDNAKNSLYLQMNSLRAEDTALYYCAKDRWDTAMITPDAFDIWGQGTMVTVSS

SEQ ID NO: 263 - protein, 118 aa, synthetic construct
  source 1..118: note = GPA33-2RmhC-22 VH
HVTLKESGGGLVKPGGSLRLSCAASGFTFSTYSMNWVRQAPGKGLEWVSSISRDSAYIYYADSVKGRFTISRDNAKNSLYLQMNSLGAEDTAVYYCVREGVAGAFDIWGQGTMVTVSS

SEQ ID NO: 264 - protein, 124 aa, synthetic construct
  source 1..124: note = GPA33-2RmhC-23 VH
QMQLVQSGGGLVQPGRSLRLSCTASGFTFGDYGMHWVRQVPGKGLEWVSGISWNSGRKGYADSVKGRFTISRDNAKNSLYLQMDSLRAEDTALYYCAKDMKIIRMEAAGPLEFWGQGTLVTVSS

SEQ ID NO: 265 - protein, 118 aa, synthetic construct
  source 1..118: note = GPA33-2RmhC-24 VH
QMQLVQSGGGLVKPGGSLRLSCAASGFTFSTYSMNWVRQAPGKGLEWVSSISRDSAYIYYADSVKGRFTISRDNAKNSLYLQMNSLRAEDTAVYYCVREGVAGAFDIWGQGTMVTVSS

SEQ ID NO: 266 - protein, 118 aa, synthetic construct
  source 1..118: note = GPA33-2RmhC-25 VH
QMQLVQSGGGLVKPGGSLRLPCAASGFTFSSYNMNWVRQAPGKGLEWVSSISSSGDFMYYADSVKGRFTISRDNAKNSLYLQMSSLRAEDTAVYYCAREGPGTPFDYWGQGTLVTVSS

SEQ ID NO: 267 - protein, 118 aa, synthetic construct
  source 1..118: note = GPA33-2RmhC-26 VH
QVTLKESGGGLVKPGGSLRLSCAASGFTFSTYSMNWVRQAPGKGLEWVSSISRDSAYIYYADSVKGRFTISRDNAKNSLYLQMNSLRAEDTAVYYCVREGVAGAFDIWGQGTMVTVSS

SEQ ID NO: 268 - protein, 124 aa, synthetic construct
  source 1..124: note = GPA33-2RmhC-27 VH
QVQLVQSGAEVKKPGSSVKVSCKASGGTFSSYAFSWVRQAPGQGLEWMGGIIPIFGTANYAQKFQDRVTITADESTSTAYMELSSLRSEDTAVYYCARAYGGSAYYHNYGMDVWGQGTTVTVSS

SEQ ID NO: 269 - protein, 122 aa, synthetic construct
  source 1..122: note = GPA33-2RmhC-28 VH
QVQLVQSGAEVKKPGASVKVSCKGSGYTFTNYGISWVRQAPGQGLEWMGWISAYNGNTNYAQKLQGRVTMTTDTSTSTVYMELRSLRSDDTAVYYCARDSPLNWGPDAFDIWGQGTMVTVSS

SEQ ID NO: 270 - protein, 123 aa, synthetic construct
  source 1..123: note = GPA33-2RmhC-29 VH
EVQLLESGPGLVKPSETLSLTCTVSGGSVSSTSYYWSWIRQPPGKGLEWIGYIYYSGSTNYNPSLKSRVTISVDTSKNQFSLKLSSMTAADTAVYYCARDRGSGWYRDAFDIWGQGTMVTVSS

SEQ ID NO: 271 - protein, 118 aa, synthetic construct
  source 1..118: note = GPA33-2RmhC-30 VH
QMQLVQSGGGLVKPGGSLRPSCAASGFTFSSYNMNWVRQAPGKGLEWVSSISSSGDFMYYADSVKGRFTISRDNAKNSLYLQMSSLRAEDTAVYYCAREGPGTPFDYWGQGTLVTVSS

SEQ ID NO: 272 - protein, 118 aa, synthetic construct
  source 1..118: note = GPA33-2RmhC-31 VH
QMQLVQSGGGLVKPGGSLRLSCAASGFTFSSYNMNWVRQAPGKGLEWVSSISSSGDFMYYADSVKGRFTISRDDAKNSLYLQMNSLRAEDTAVYYCAREGPGTPFDYWGQGTLVTVSS

SEQ ID NO: 273 - protein, 122 aa, synthetic construct
  source 1..122: note = GPA33-2RmhC-32 VH
EVQLVESGGGLVQPGRSLRLSCAASGFTFDDYAMHWVRQAPGKGLEWVSGISWSSGSIGYADSVKGRFTISRDNAKSSLYLQMNSLRAEDTALYYCAKDITDSSGYYGMDAWGQGTLVTVSS

SEQ ID NO: 274 - protein, 118 aa, synthetic construct
  source 1..118: note = GPA33-2RmhC-33 VH
QMQLVQSGGGLVKPGGSLRLSCAAPGFTFSSYNMNWVRQAPGKGLEWVSSISSSGDFMYYADSVKGRFTISRDNAKNSLYLQMSSLRAEDTAVYYCAREGPGTPFDYWGQGTLVTVSS

SEQ ID NO: 275 - protein, 118 aa, synthetic construct
  source 1..118: note = GPA33-2RmhC-34 VH
QVQLVQSGGGLVKSGGSLRLSCAASGFTFSNYNMNWVRQAPGKGLEWVSSISSSGDFMYYADSVKGRFTISRDDAKNSLYLQMNSLRAEDTAVYYCAREGPGTPFDYWGQGTLVTVSS

SEQ ID NO: 276 - protein, 118 aa, synthetic construct
  source 1..118: note = GPA33-2RmhC-35 VH
QMQLVQSGGGLVKPGGSLRLSCAASGFTFSSYNMNWVRQAPGKGLEWVSSISSSGDFMYYADSVKGRFTISRDNAKNSLYLQMSSLRAEDTAVYYCAREGPGTPLDYWGQGTLVTVSS

SEQ ID NO: 277 - protein, 118 aa, synthetic construct
  source 1..118: note = GPA33-2RmhC-36 VH
QVQLQESGGGLVKPGGSLRLSCAASGFTFSNFNMNWVRQAPGKGLEWVSSISSSGDFMYYADSVKGRFTISRDNAKNSLYLQMNSLRAEDTAVYYCAREGPGTPFDYWGQGTLVTVSS

SEQ ID NO: 278 - protein, 124 aa, synthetic construct
  source 1..124: note = GPA33-2RmhC-37 VH
QVQLVESGPGLVKPSETLSLTCTVSGGSISSYYWSWIRQPPGKGLEWIGYIYHSGSTNYNPSLKSRVTISVDTSKNQFSLKLSSVTAADTAVYYYARSRQQLLRDYYYYGMDVWGQGTTVTVST

SEQ ID NO: 279 - protein, 118 aa, synthetic construct
  source 1..118: note = GPA33-2RmhC-38 VH
QMQLVQSGGGLVKPGGSLRLSCAASGFTFSSYNMNWVRQAPGKGLEWVSSISSSGDFMYYADSVKGRFTISRGNAKNSLYLQMSSLRAEDTAVYYCAREGPGTPFDYWGQGTLVTVSS

SEQ ID NO: 280 - protein, 118 aa, synthetic construct
  source 1..118: note = GPA33-2RmhC-39 VH
QMQLVQSGGGLVKPGGSLRLSCAASGFTFSSYNMNWVRQAPGKGLEWVSSISSSGDYMYYADSVKGRFTISRDNAKNSLYLQMNSLRAEDTAVYYCAREGPGTPFDYWGQGTLVTVSS

SEQ ID NO: 281 - protein, 126 aa, synthetic construct
  source 1..126: note = GPA33-2RmhC-40 VH
EVQLVESGGGLAQPGGSLRLSCAASGFTFSNYAMSWVRQAPGKGLEWVSAISGSGGSTYYADSVKGRFTISRDNSKNTLYLQMNSLRAEDTAVYYCAKGSGSYYKPVYYYYGMDVWGQGTTVTVSS

SEQ ID NO: 282 - protein, 118 aa, synthetic construct
  source 1..118: note = GPA33-2RmhC-41 VH
QVQLVQSGGGLVKPGGSLRLSCAASGFTFSNYNMNWVRQAPGKGLEWVSSISSSGDFMYYADSVKGRFTISRDDAKNSLYLQMNSLRAEDTAVYYCAREGPGTPFDYWGQGTLVIVSS

SEQ ID NO: 283 - protein, 121 aa, synthetic construct
  source 1..121: note = GPA33-2RmhC-42 VH
EVQLVESGGGLVQPGRSLRLSCAASGFTFDDYAMHWVRQAPGKGLEWVSGISWNSGSIGYADSVKGRFTISRDNAKNSLYLQMNSLRAEDTALYYCAKCDGSGSYGAFDIWGQGTMVTVSS

SEQ ID NO: 284 - protein, 126 aa, synthetic construct
  source 1..126: note = GPA33-2RmhC-43 VH
QVQLVQSGAEVKKPGSSVKVSCKASGGTFSSYAISWVRQAPGQGLEWMGGIIPIFGTANYAQKFQGRVTITADESTSTAYMELSSLRSEDTAVYYCARAPDILTSSGYYYYGMDVWGQGTTVTASS

SEQ ID NO: 285 - protein, 120 aa, synthetic construct
  source 1..120: note = GPA33-2RmhC-44 VH
QVQLVQSGAEVKKPGASVKVSCKVSGYTLTELSMHWVRQAPGKGLEWMGGFDPEDGETIYAQKFQGRVTMTEDTSTDTAYMELSSLRSEDTAVYYCATEAAAGTPFFDYWGQGTLVTASS

SEQ ID NO: 286 - protein, 123 aa, synthetic construct
  source 1..123: note = GPA33-2RmhC-45 VH
QLQLQESGPGLVKPSETLSLTCTVSGGSVTSTSYYWSWIRQPPGKGLEWIGYIYYSGSTNYNPSLKSRVTISVDTSKNQFSLKLSSVTAADTAVYYCARDRGSGWYRDAFDIWGQGTMVTVSS

SEQ ID NO: 287 - protein, 121 aa, synthetic construct
  source 1..121: note = GPA33-2RmhC-46 VH
QVTLKESGGGLVQPGRSLRLSCAASGFTFDDYAMHWVRQAPGKGLEWVSGISWNSGSIGYADSVKGRFTISRDNAKNSLYLQMNSLRAEDTALYYCAKDIGAVAGYGMDVWGQGTTVTVSS

SEQ ID NO: 288 - protein, 123 aa, synthetic construct
  source 1..123: note = GPA33-2RmhC-47 VH
QVQLQESGPGLVKPSQTLSFTCAISGDSVSSNSAAWNWIRQSPSRGLEWLGRTYYRSKWYNDYALSVKSRITINPDTSKNQFSLHLNSVTPEDTAVYYCAREKTGLYWYFDLWGRGTLVTVSS

SEQ ID NO: 289 - protein, 124 aa, synthetic construct
  source 1..124: note = GPA33-2RmhC-48 VH
QVQLVQSGAEVKKPGSSVKVSCKASGGTFNTYAINWVRQAPGQGLEWMGGIIPIFGSANYAQKFQDRVTITADESTSTAYMELSSLRSEDTAVYYCARAYGGSAHYYSYGMDVWGQGTLVTVSS

SEQ ID NO: 290 - protein, 126 aa, synthetic construct
  source 1..126: note = GPA33-2RmhC-49 VH
EVQLVESGGGLVQPGGSLRLSCAASGFTFSSYGMNWVRQAPGKGLEWVSYISTSSSSIYYADSVKGRFTISRDNAKNSLYLQMNSLRDEDTAVYYCARDGAYCGGDCYPYWNFDLWGHGTLVTVSS

SEQ ID NO: 291 - protein, 117 aa, synthetic construct
  source 1..117: note = GPA33-2RmhC-50 VH
EVQLVESGAEVKKPGESLKISCKGSGYSFTDSWIGWVRQMPGKGLEWMGIIYPGDSDTRYSPSFQGQVTTSADKSISTAYLQWSSLKASDTAMYYCARPYRDYSFDYWGQGPWSPSR

SEQ ID NO: 292 - DNA, 1470 bp, synthetic construct
  source 1..1470: mol_type = other DNA; note = Cont-scFv-Fc
atgtacaggatgcaactcctgtcttgcattgcactaagtcttgcacttgtcacgaattcggaggtgcaattgttggagtctgggggaggcttggtacagcctggggggtccctgagactctcctgtgcagcctccggattcacctttagcagttatgccatgagctgggtccgccaggctccagggaaggggctggagtgggtctcagctattagtggtagtggtggtagcacatactacgcagactccgtgaagggccggttcaccatctccagagacaattccaagaacacgctgtatctgcagatgaacagcctgagagccgaggacacggccgtatattactgtgcgaaaggcagcggatttgactactggggccaaggaaccctggtcaccgtctcgagtggtggaggcggttcaggcggaggtggctctgggtcgacgggatcggaaatcgtgttaacgcagtctccaggcaccctgtctttgtctccaggggaaagagccaccctctcttgcagggccagtcagagtgttagcagcagctacttagcctggtaccagcagaaacctggccaggctcccaggctcctcatctatggagcatccagcagggccactggcatcccagacaggttcagtggcagtggatccgggacagacttcactctcaccatcagcagactggagcctgaagattttgcagtgtattactgtcagcagtatggtagctcaccgctgacgttcggccaggggaccaaagtggaaatcaaacccaaatctagcgacaaaactcacacatgcccaccgtgcccagcacctgaagccgagggggccccgtcagtcttcctcttccccccaaaacccaaggacaccctcatgatctcccggacccctgaggtcacatgcgtggtggtggacgtgagccacgaagaccctgaggtcaagttcaactggtacgtggacggcgtggaggtgcataatgccaagacaaagccgcgggaggagcagtacaacagcacgtaccgtgtggtcagcgtcctcaccgtcctgcaccaggactggctgaatggcaaggagtacaagtgcgccgtctccaacaaagccctcccagcctccatcgagaaaaccatctccaaagccaaagggcagccccgagaaccacaggtgtacaccctgcccccatcccgggaggagatgaccaagaaccaggtcagcctgacctgcctggtcaaaggcttctatcccagcgacatcgccgtggagtgggagagcaatgggcagccggagaacaactacaagaccacgcctcccgtgctggactccgacggctccttcttcctctatagcaagctcaccgtggacaagagcaggtggcagcaggggaacgtcttctcatgctccgtgatgcatgaggctctgcacaaccactacacgcagaagagcctctccctgtccccgggtaaatag

SEQ ID NO: 293 - DNA, 1155 bp, synthetic construct
  source 1..1155: mol_type = other DNA; note = R1CRD-Fc
atgcgtctgggcctctgtgtcgttgccttggtgctgagttggacgcatctgaccattagctctcgagggattaagggcaaacgccaaaggaggataagcgccgaagggagccaggcttgtgccaagggatgcgagctgtgtagcgaggtgaacggatgtttgaaatgtagccccaaactgttcattctgctggaacggaacgacatcagacaggttggcgtctgtctgccctcatgtccaccaggctattttgatgctcggaaccccgacatgaacaagtgcatcaagtgcaagatagagcattgcgaagcctgtttcagtcacaacttctgcactaagtgcaaggaaggactgtatctgcacaaaggcagatgctatcctgcgtgtccggagggttccagcgctgcaaatggaaccatggagtgctcttcccctgcatccacaactgagaatctctattttcagggtagcactgggacacacacttgccctccctgccccgctcccgaagcagaaggtgcgccatctgtctttctctttccacccaaaccaaaagacacactcatgatctctcgcacacccgaagtcacctgtgtggtcgtagacgtttcacatgaggacccagaggtgaagttcaactggtatgtggatggggtggaggtacacaatgcaaagaccaaaccacgcgaagagcagtacaatagcacttacagagtggtgtcagtgctcaccgttttgcatcaggattggctgaatggtaaggagtacaagtgcgccgtgtccaataaggccttgcctgcaagcatcgagaaaaccatctcaaaggccaaaggacaaccgagggagcctcaggtttatacccttcctcccagtcgagaggaaatgacgaagaaccaggtcagtcttacatgcctggtaaagggcttttacccttctgacattgccgtggaatgggagtcaaatggccagcccgagaacaactacaagactacgccgccagtcctggatagcgatggatccttcttcctgtactccaaactgacagtggataaatctcggtggcagcaaggcaatgtgtttagctgcagtgtgatgcacgaagctctgcacaaccattacacccagaaatccctttccctttctcctgggaaatga

SEQ ID NO: 294 - DNA, 1128 bp, synthetic construct
  source 1..1128: mol_type = other DNA; note = R4CRD-Fc
atgagagctcccttgtgtctcctgctgttggttgcacatgccgtggatatgcttgccctgaatcggaggaagaaacaggtcggaactggccttggtgggaactgtactggctgcatcatctgcagcgaggagaatggatgttccacatgccagcaaaggctcttcctgtttatccgaagggagggtatacgccagtatgggaagtgcctgcacgattgcccacccggatacttcggcattagaggacaggaagtgaaccgttgcaagaaatgtggggcgacttgtgaatcttgcttctcccaggacttctgcattcggtgcaagagacagttttacctctacaaaggcaaatgcctgcccacatgtccgccgggtacacttgcccaccagaatactagggaatgtcaaggcagcacgaccgagaacctgtattttcagggctctactgggactcacacgtgtcctccatgcccagctccagaggcagaaggagcaccttcagtgtttctctttccacccaagcccaaggacaccctgatgatctcaagaacccctgaggttacatgcgtggttgtggatgtgtcacacgaggatccggaggtcaaattcaactggtacgtagacggggtcgaggttcacaatgccaagacaaagcctcgcgaagagcagtacaacagcacctatcgcgtggtgagtgtcctgaccgtactgcatcaagactggctgaatggcaaggagtataagtgtgcggtgtctaacaaagctcttcccgcaagcatagaaaagaccatctccaaagccaaaggtcaacctcgggaacctcaggtctatacactgccaccctcacgggaagaaatgacgaagaatcaggtgtctctgacttgtctggtgaagggcttctaccctagcgacattgccgtggagtgggagagtaatgggcagcccgagaacaactacaagacaaccccacctgttctggatagtgatggcagcttcttcttgtactccaaattgaccgtagacaaatcccgatggcaacagggaaatgtctttagctgcagcgtgatgcatgaagctctccataaccactatacccagaagtccctgagtctctctcccggaaaatag

SEQ ID NO: 295 - DNA, 1476 bp, synthetic construct
  source 1..1476: mol_type = other DNA; note = GPA2RC9-scFv-Fc
atgtacagaatgcagctgctgagctgtatcgccctgtctctggccctggtcaccaattctcaggtgcagctggttcagtctggcggcggacttgtgaaacctggcggaagcctgagactgagctgtgccgcttccggcttcaccttcagcaactacaacatgaactgggtccgacaggcccctggcaaaggccttgaatgggtgtccagcatcagcagcagcggcgacttcatgtactacgccgacagcgtgaagggcagattcaccatcagcagggacgacgccaagaacagcctgtacctgcagatgaactccctgagagccgaggacaccgccgtgtactactgtgccagagaaggccctggcacacccttcgattattggggccagggcacactggtcaccgtttctagcggaggcggaggatcaggtggtggcggatctggatctacaggcagcgccatccagatgacacagagcccttctagcctgagcgccagcgtgggagacagagtgaccatcacatgtagagccagccagagcatcagctcctacctgaactggtatcagcagaagcccggcaaggcccctaagctgctgatctatgctgccagctctctgcagtccggcgtgccatctagattttctggctctggcagcggcaccgacttcaccctgaccatatctagcctgcagcctgaggacttcgccacctactactgccagcagagctacagaaccccttacaccttcggacagggcaccaaggtggaaatcaagcccaagagcagcgacaagacccacacctgtcctccatgtcctgctccagaagctgaaggcgccccttccgtgttcctgtttcctccaaagcctaaggacaccctgatgatcagcaggacccctgaagtgacctgcgtggtggtggatgtgtcccacgaggatcccgaagtgaagttcaattggtacgtggacggcgtggaagtgcacaacgccaagaccaagcctagagaggaacagtacaacagcacctacagagtggtgtccgtgctgaccgtgctgcaccaggattggctgaacggcaaagagtacaagtgcgccgtgtccaacaaagccctgcctgccagcatcgagaaaaccatctccaaggccaagggccagcctagggaaccccaggtttacacactgcctccaagccgggaagagatgaccaagaaccaggtgtccctgacctgcctggtcaagggcttctacccttccgatatcgccgtggaatgggagagcaatggccagcctgagaacaactacaagacaacccctcctgtgctggacagcgacggctcattcttcctgtacagcaagctgacagtggacaagagcagatggcagcagggcaacgtgttcagctgcagcgtgatgcacgaggccctgcacaaccactacacccagaagtctctgagcctgtctcctggcaagtga

SEQ ID NO: 296 - DNA, 1476 bp, synthetic construct
  source 1..1476: mol_type = other DNA; note = GPA2RC17-scFv-Fc
atgtacagaatgcagctgctgagctgtatcgccctgtctctggccctggtcaccaactctcagatgcagctggttcagtctggcggcggacttgtgaaacctggcggaagcctgagactgagctgtgccgcttccggcttcaccttcagcagctacaacatgaactgggtccgacaggcccctggcaaaggccttgaatgggtgtccagcatcagcagcagcggcgacttcatgtactacgccgacagcgtgaagggcagattcaccatctccagagacaacgccaagaacagcctgtacctgcagatgagcagcctgagagccgaggataccgccgtgtactactgcgccagagaaggccctggcacaccctttgattattggggccagggcacactggtcaccgtttctagcggaggcggaggatcaggtggtggcggatctggatctacaggctctgccatccagctgacacagagcccttctagcctgtctgccagcgtgggcgacagagtgaccatcacatgtagagccagccagagcatctccagctttctgaactggtatcagcacaagcccggcaaggcccctaagctgctgatctatgtggccagctctctgcagtccggcgtgccatctagattttctggcagcggctccggcaccgacttcaccctgacaatatctagcctgcagccagaggacttcgccacctactactgtcagcagagccacaacaccccttacaccttcggacagggcaccaagctggaaatcaagcccaagagcagcgacaagacccacacctgtcctccatgtcctgctccagaagctgaaggcgccccttccgtgttcctgtttcctccaaagcctaaggacaccctgatgatcagcagaacccctgaagtgacctgcgtggtggtggatgtgtcccacgaggatcccgaagtgaagttcaattggtacgtggacggcgtggaagtgcacaatgccaagaccaagcctagagaggaacagtacaacagcacctacagagtggtgtccgtgctgaccgtgctgcaccaggattggctgaacggcaaagagtacaagtgcgccgtgtccaacaaagccctgcctgccagcatcgagaaaaccatcagcaaggccaagggccagcctagggaaccccaggtttacacactgcctccaagccgggaagagatgaccaagaaccaggtgtccctgacctgcctggtcaagggcttctacccttccgatatcgccgtggaatgggagagcaatggacagcccgagaacaactacaagacaacccctcctgtgctggacagcgacggctcattcttcctgtacagcaagctgacagtggacaagagcagatggcagcagggcaacgtgttcagctgcagcgtgatgcacgaggccctgcacaaccactacacccagaagtctctgagcctgtctcctggcaagtga

SEQ ID NO: 297 - DNA, 1473 bp, synthetic construct
  source 1..1473: mol_type = other DNA; note = GPA2RC28-scFv-Fc
atgtacagaatgcagctgctgagctgtatcgccctgtctctggccctggtcaccaattctgaggtgcagctggtggaatctggcggcggacttgtgaaacctggcggctctctgagactgagctgtgccgcttccggcttcaccttcagcagctacagcatgaactgggtccgacaggcccctggcaaaggccttgaatgggtgtccagcatcagccgggacagcacctacatctactacgccgacagcgtgaagggcagattcaccatctccagagacaacgccaagaacagcctgtacctgcagatgaactccctgagagccgaggacaccgccgtgtactactgtgctagagaaggcgtggcaggcgccttcgatatttggggccagggcacaatggtcaccgtgtctagcggaggcggaggatcaggtggtggtggatctggatctacaggcagcgccatccagctgacacagagccctagtagcctgtctgccagcgtgggcgacagagtgaccatcacatgtagagccagccagagcatcagctcctacctgaactggtatcagcagaagcccggcaaggcccctaagctgctgatctacattgccagcagcctgcagagcggcgtgccaagcagattttctggcagcggctctggcaccgacttcaccctgaccatatctagcctgcagcctgaggacttcgccacctactactgccagcagagctacaacacctggaccttcggacagggcaccaaggtggaaatcaagcccaagagcagcgacaagacccacacctgtcctccatgtcctgctccagaagctgaaggcgccccttccgtgttcctgtttcctccaaagcctaaggacaccctgatgatcagcaggacccctgaagtgacctgcgtggtggtcgatgtgtcccacgaggatcccgaagtgaagttcaattggtacgtggacggcgtggaagtgcacaatgccaagaccaagcctagagaggaacagtacaactccacctacagagtggtgtccgtgctgaccgtgctgcaccaggattggctgaacggcaaagagtacaagtgcgccgtgtccaacaaagccctgcctgccagcatcgagaaaaccatcagcaaggccaagggccagcctagggaaccccaggtttacacactgcctccaagccgggaagagatgaccaagaaccaggtgtccctgacctgcctggtcaagggcttctacccttccgatatcgccgtggaatgggagagcaatggccagcctgagaacaactacaagacaacccctcctgtgctggacagcgacggctcattcttcctgtacagcaagctgacagtggacaagagcagatggcagcagggcaacgtgttcagctgcagcgtgatgcacgaggccctgcacaaccactacacccagaagtctctgagcctgtctcctggcaagtga

SEQ ID NO: 298 - DNA, 1512 bp, synthetic construct
  source 1..1512: mol_type = other DNA; note = Rspo1FL-Fc
gccaccatgcggcttgggctgtgtgtggtggccctggttctgagctggacgcacctcaccatcagcagccgggggatcaaggggaaaaggcagaggcggatcagtgccgaggggagccaggcctgtgccaaaggctgtgagctctgctctgaagtcaacggctgcctcaagtgctcacccaagctgttcatcctgctggagaggaacgacatccgccaggtgggcgtctgcttgccgtcctgcccacctggatacttcgacgcccgcaaccccgacatgaacaagtgcatcaaatgcaagatcgagcactgtgaggcctgcttcagccataacttctgcaccaagtgtaaggagggcttgtacctgcacaagggccgctgctatccagcttgtcccgagggctcctcagctgccaatggcaccatggagtgcagtagtcctgcgcaatgtgaaatgagcgagtggtctccgtgggggccctgctccaagaagcagcagctctgtggtttccggaggggctccgaggagcggacacgcagggtgctacatgcccctgtgggggaccatgctgcctgctctgacaccaaggagacccggaggtgcacagtgaggagagtgccgtgtcctgaggggcagaagaggaggaagggaggccagggccggcgggagaatgccaacaggaacctggccaggaaggagagcaaggaggcgggtgctggctctcgaagacgcaaggggcagcaacagcagcagcagcaagggacagtggggccactcacatctgcagggcctgccagcactactgagaatctttattttcagggatcaaccggcactcacacatgcccaccgtgcccagcacctgaagccgagggggccccgtcagtcttcctcttccccccaaaacccaaggacaccctcatgatctcccggacccctgaggtcacatgcgtggtggtggacgtgagccacgaagaccctgaggtcaagttcaactggtacgtggacggcgtggaggtgcataatgccaagacaaagccgcgggaggagcagtacaacagcacgtaccgtgtggtcagcgtcctcaccgtcctgcaccaggactggctgaatggcaaggagtacaagtgcgccgtctccaacaaagccctcccagcctccatcgagaaaaccatctccaaagccaaagggcagccccgagaaccacaggtgtacaccctgcccccatcccgggaggagatgaccaagaaccaggtcagcctgacctgcctggtcaaaggcttctatcccagcgacatcgccgtggagtgggagagcaatgggcagccggagaacaactacaagaccacgcctcccgtgctggactccgacggctccttcttcctctatagcaagctcaccgtggacaagagcaggtggcagcaggggaacgtcttctcatgctccgtgatgcatgaggctctgcacaaccactacacgcagaagagcctctccctgtccccgggtaaatga

SEQ ID NO: 299 - DNA, 1470 bp, synthetic construct
  source 1..1470: mol_type = other DNA; note = Cont-scFv-Fc-Knob
atgtacaggatgcaactcctgtcttgcattgcactaagtcttgcacttgtcacgaattcggaggtgcaattgttggagtctgggggaggcttggtacagcctggggggtccctgagactctcctgtgcagcctccggattcacctttagcagttatgccatgagctgggtccgccaggctccagggaaggggctggagtgggtctcagctattagtggtagtggtggtagcacatactacgcagactccgtgaagggccggttcaccatctccagagacaattccaagaacacgctgtatctgcagatgaacagcctgagagccgaggacacggccgtatattactgtgcgaaaggcagcggatttgactactggggccaaggaaccctggtcaccgtctcgagtggtggaggcggttcaggcggaggtggctctgggtcgacgggatcggaaatcgtgttaacgcagtctccaggcaccctgtctttgtctccaggggaaagagccaccctctcttgcagggccagtcagagtgttagcagcagctacttagcctggtaccagcagaaacctggccaggctcccaggctcctcatctatggagcatccagcagggccactggcatcccagacaggttcagtggcagtggatccgggacagacttcactctcaccatcagcagactggagcctgaagattttgcagtgtattactgtcagcagtatggtagctcaccgctgacgttcggccaggggaccaaagtggaaatcaaacccaaatctagcgacaaaactcacacatgcccaccgtgcccagcacctgaagccgagggggccccgtcagtcttcctcttccccccaaaacccaaggacaccctcatgatctcccggacccctgaggtcacatgcgtggtggtggacgtgagccacgaagaccctgaggtcaagttcaactggtacgtggacggcgtggaggtgcataatgccaagacaaagccgcgggaggagcagtacaacagcacgtaccgtgtggtcagcgtcctcaccgtcctgcaccaggactggctgaatggcaaggagtacaagtgcgccgtctccaacaaagccctcccagcctccatcgagaaaaccatctccaaagccaaagggcagccccgagaaccacaggtgtacaccctgcccccatgccgggaggagatgaccaagaaccaggtcagcctgtggtgcctggtcaaaggcttctatcccagcgacatcgccgtggagtgggagagcaatgggcagccggagaacaactacaagaccacgcctcccgtgctggactccgacggctccttcttcctctatagcgcgctcaccgtggacaagagcaggtggcagcaggggaacgtcttctcatgctccgtgatgcatgaggctctgcacaaccactacacgcagaagagcctctccctgtccccgggtaaatag

SEQ ID NO: 300 - DNA, 1470 bp, synthetic construct
  source 1..1470: mol_type = other DNA; note = Cont-scFv-Fc-Hole
atgtacaggatgcaactcctgtcttgcattgcactaagtcttgcacttgtcacgaattcggaggtgcaattgttggagtctgggggaggcttggtacagcctggggggtccctgagactctcctgtgcagcctccggattcacctttagcagttatgccatgagctgggtccgccaggctccagggaaggggctggagtgggtctcagctattagtggtagtggtggtagcacatactacgcagactccgtgaagggccggttcaccatctccagagacaattccaagaacacgctgtatctgcagatgaacagcctgagagccgaggacacggccgtatattactgtgcgaaaggcagcggatttgactactggggccaaggaaccctggtcaccgtctcgagtggtggaggcggttcaggcggaggtggctctgggtcgacgggatcggaaatcgtgttaacgcagtctccaggcaccctgtctttgtctccaggggaaagagccaccctctcttgcagggccagtcagagtgttagcagcagctacttagcctggtaccagcagaaacctggccaggctcccaggctcctcatctatggagcatccagcagggccactggcatcccagacaggttcagtggcagtggatccgggacagacttcactctcaccatcagcagactggagcctgaagattttgcagtgtattactgtcagcagtatggtagctcaccgctgacgttcggccaggggaccaaagtggaaatcaaacccaaatctagcgacaaaactcacacatgcccaccgtgcccagcacctgaagccgagggggccccgtcagtcttcctcttccccccaaaacccaaggacaccctcatgatctcccggacccctgaggtcacatgcgtggtggtggacgtgagccacgaagaccctgaggtcaagttcaactggtacgtggacggcgtggaggtgcataatgccaagacaaagccgcgggaggagcagtacaacagcacgtaccgtgtggtcagcgtcctcaccgtcctgcaccaggactggctgaatggcaaggagtacaagtgcgccgtctccaacaaagccctcccagcctccatcgagaaaaccatctccaaagccaaagggcagccccgagaaccacaggtgtgcaccctgcccccatcccgggaggagatgaccaagaaccaggtcagcctgtcctgcgcggtcaaaggcttctatcccagcgacatcgccgtggagtgggagagcaatgggcagccggagaacaactacaagaccacgcctcccgtgctggactccgacggctccttcaaactcgttagcaagctcaccgtggacaagagcaggtggcagcaggggaacgtcttctcatgctccgtgatgcatgaggctctgcacaaccactacacgcagaagagcctctccctgtccccgggtaaatag

SEQ ID NO: 301 - DNA, 1155 bp, synthetic construct
  source 1..1155: mol_type = other DNA; note = Rspo1CRD-scFv-Fc-Knob
atgcgtctgggcctctgtgtcgttgccttggtgctgagttggacgcatctgaccattagctctcgagggattaagggcaaacgccaaaggaggataagcgccgaagggagccaggcttgtgccaagggatgcgagctgtgtagcgaggtgaacggatgtttgaaatgtagccccaaactgttcattctgctggaacggaacgacatcagacaggttggcgtctgtctgccctcatgtccaccaggctattttgatgctcggaaccccgacatgaacaagtgcatcaagtgcaagatagagcattgcgaagcctgtttcagtcacaacttctgcactaagtgcaaggaaggactgtatctgcacaaaggcagatgctatcctgcgtgtccggagggttccagcgctgcaaatggaaccatggagtgctcttcccctgcatccacaactgagaatctctattttcagggtagcactgggacacacacttgccctccctgcccagcacctgaagccgagggggccccgtcagtcttcctcttccccccaaaacccaaggacaccctcatgatctcccggacccctgaggtcacatgcgtggtggtggacgtgagccacgaagaccctgaggtcaagttcaactggtacgtggacggcgtggaggtgcataatgccaagacaaagccgcgggaggagcagtacaacagcacgtaccgtgtggtcagcgtcctcaccgtcctgcaccaggactggctgaatggcaaggagtacaagtgcgccgtctccaacaaagccctcccagcctccatcgagaaaaccatctccaaagccaaagggcagccccgagaaccacaggtgtacaccctgcccccatgccgggaggagatgaccaagaaccaggtcagcctgtggtgcctggtcaaaggcttctatcccagcgacatcgccgtggagtgggagagcaatgggcagccggagaacaactacaagaccacgcctcccgtgctggactccgacggctccttcttcctctatagcgcgctcaccgtggacaagagcaggtggcagcaggggaacgtcttctcatgctccgtgatgcatgaggctctgcacaaccactacacgcagaagagcctctccctgtccccgggtaaatag

SEQ ID NO: 302 - DNA, 1155 bp, synthetic construct
  source 1..1155: mol_type = other DNA; note = Rspo1CRD-scFv-Fc-Hole
atgcgtctgggcctctgtgtcgttgccttggtgctgagttggacgcatctgaccattagctctcgagggattaagggcaaacgccaaaggaggataagcgccgaagggagccaggcttgtgccaagggatgcgagctgtgtagcgaggtgaacggatgtttgaaatgtagccccaaactgttcattctgctggaacggaacgacatcagacaggttggcgtctgtctgccctcatgtccaccaggctattttgatgctcggaaccccgacatgaacaagtgcatcaagtgcaagatagagcattgcgaagcctgtttcagtcacaacttctgcactaagtgcaaggaaggactgtatctgcacaaaggcagatgctatcctgcgtgtccggagggttccagcgctgcaaatggaaccatggagtgctcttcccctgcatccacaactgagaatctctattttcagggtagcactgggacacacacttgccctccctgcccagcacctgaagccgagggggccccgtcagtcttcctcttccccccaaaacccaaggacaccctcatgatctcccggacccctgaggtcacatgcgtggtggtggacgtgagccacgaagaccctgaggtcaagttcaactggtacgtggacggcgtggaggtgcataatgccaagacaaagccgcgggaggagcagtacaacagcacgtaccgtgtggtcagcgtcctcaccgtcctgcaccaggactggctgaatggcaaggagtacaagtgcgccgtctccaacaaagccctcccagcctccatcgagaaaaccatctccaaagccaaagggcagccccgagaaccacaggtgtgcaccctgcccccatcccgggaggagatgaccaagaaccaggtcagcctgtcctgcgcggtcaaaggcttctatcccagcgacatcgccgtggagtgggagagcaatgggcagccggagaacaactacaagaccacgcctcccgtgctggactccgacggctccttcaaactcgttagcaagctcaccgtggacaagagcaggtggcagcaggggaacgtcttctcatgctccgtgatgcatgaggctctgcacaaccactacacgcagaagagcctctccctgtccccgggtaaatag

SEQ ID NO: 303 - DNA, 1476 bp, synthetic construct
  source 1..1476: mol_type = other DNA; note = GPARC12-scFv-Fc-Knob
atgtacagaatgcagctgctgagctgtatcgccctgtctctggccctggtcaccaattctcaggtgcagctggttcagtctggcggcggacttgtgaaacctggcggaagcctgagactgagctgtgccgcttccggcttcaccttcagcaactacaacatgaactgggtccgacaggcccctggcaaaggccttgaatgggtgtccagcatcagcagcagcggcgacttcatgtactacgccgacagcgtgaagggcagattcaccatcagcagggacgacgccaagaacagcctgtacctgcagatgaactccctgagagccgaggacaccgccgtgtactactgtgccagagaaggccctggcacacccagcgattattggggacagggcacactggtcaccgtgtctagcggaggcggaggatcaggtggtggtggatctggctctacaggcagcgccatccagatgacacagagcccctctagcctgtacgccagcgtgggagacagagtgaccatcacatgcagagccagccagagcatcagctcctacctgaactggtatcagcagaagcccggcaaggcccctaagctgctgatctacgatgccagctctctgcagtccggcgtgccaagcagattttctggcagcggctctggcaccgacttcaccctgaccatatctagcctgcagcctgaggacttcgccacctactactgccagcagagctacagaaccccttacacctttggccagggcaccaaggtggaaatcaagcccaaatctagcgacaaaactcacacatgcccaccgtgcccagcacctgaagccgagggggccccgtcagtcttcctcttccccccaaaacccaaggacaccctcatgatctcccggacccctgaggtcacatgcgtggtggtggacgtgagccacgaagaccctgaggtcaagttcaactggtacgtggacggcgtggaggtgcataatgccaagacaaagccgcgggaggagcagtacaacagcacgtaccgtgtggtcagcgtcctcaccgtcctgcaccaggactggctgaatggcaaggagtacaagtgcgccgtctccaacaaagccctcccagcctccatcgagaaaaccatctccaaagccaaagggcagccccgagaaccacaggtgtacaccctgcccccatgccgggaggagatgaccaagaaccaggtcagcctgtggtgcctggtcaaaggcttctatcccagcgacatcgccgtggagtgggagagcaatgggcagccggagaacaactacaagaccacgcctcccgtgctggactccgacggctccttcttcctctatagcgcgctcaccgtggacaagagcaggtggcagcaggggaacgtcttctcatgctccgtgatgcatgaggctctgcacaaccactacacgcagaagagcctctccctgtccccgggtaaatag

SEQ ID NO: 304 - DNA, 1476 bp, synthetic construct
  source 1..1476: mol_type = other DNA; note = GPARC12-scFv-Fc-Hole
atgtacagaatgcagctgctgagctgtatcgccctgtctctggccctggtcaccaattctcaggtgcagctggttcagtctggcggcggacttgtgaaacctggcggaagcctgagactgagctgtgccgcttccggcttcaccttcagcaactacaacatgaactgggtccgacaggcccctggcaaaggccttgaatgggtgtccagcatcagcagcagcggcgacttcatgtactacgccgacagcgtgaagggcagattcaccatcagcagggacgacgccaagaacagcctgtacctgcagatgaactccctgagagccgaggacaccgccgtgtactactgtgccagagaaggccctggcacacccagcgattattggggacagggcacactggtcaccgtgtctagcggaggcggaggatcaggtggtggtggatctggctctacaggcagcgccatccagatgacacagagcccctctagcctgtacgccagcgtgggagacagagtgaccatcacatgcagagccagccagagcatcagctcctacctgaactggtatcagcagaagcccggcaaggcccctaagctgctgatctacgatgccagctctctgcagtccggcgtgccaagcagattttctggcagcggctctggcaccgacttcaccctgaccatatctagcctgcagcctgaggacttcgccacctactactgccagcagagctacagaaccccttacacctttggccagggcaccaaggtggaaatcaagcccaaatctagcgacaaaactcacacatgcccaccgtgcccagcacctgaagccgagggggccccgtcagtcttcctcttccccccaaaacccaaggacaccctcatgatctcccggacccctgaggtcacatgcgtggtggtggacgtgagccacgaagaccctgaggtcaagttcaactggtacgtggacggcgtggaggtgcataatgccaagacaaagccgcgggaggagcagtacaacagcacgtaccgtgtggtcagcgtcctcaccgtcctgcaccaggactggctgaatggcaaggagtacaagtgcgccgtctccaacaaagccctcccagcctccatcgagaaaaccatctccaaagccaaagggcagccccgagaaccacaggtgtgcaccctgcccccatcccgggaggagatgaccaagaaccaggtcagcctgtcctgcgcggtcaaaggcttctatcccagcgacatcgccgtggagtgggagagcaatgggcagccggagaacaactacaagaccacgcctcccgtgctggactccgacggctccttcaaactcgttagcaagctcaccgtggacaagagcaggtggcagcaggggaacgtcttctcatgctccgtgatgcatgaggctctgcacaaccactacacgcagaagagcctctccctgtccccgggtaaatag

SEQ ID NO: 305 - DNA, 1476 bp, synthetic construct
  source 1..1476: mol_type = other DNA; note = GPARC17-scFv-Fc-Knob
atgtacagaatgcagctgctgagctgtatcgccctgtctctggccctggtcaccaactctcagatgcagctggttcagtctggcggcggacttgtgaaacctggcggaagcctgagactgagctgtgccgcttccggcttcaccttcagcagctacaacatgaactgggtccgacaggcccctggcaaaggccttgaatgggtgtccagcatcagcagcagcggcgacttcatgtactacgccgacagcgtgaagggcagattcaccatctccagagacaacgccaagaacagcctgtacctgcagatgagcagcctgagagccgaggataccgccgtgtactactgcgccagagaaggccctggcacaccctttgattattggggccagggcacactggtcaccgtttctagcggaggcggaggatcaggtggtggcggatctggatctacaggctctgccatccagctgacacagagcccttctagcctgtctgccagcgtgggcgacagagtgaccatcacatgtagagccagccagagcatctccagctttctgaactggtatcagcacaagcccggcaaggcccctaagctgctgatctatgtggccagctctctgcagtccggcgtgccatctagattttctggcagcggctccggcaccgacttcaccctgacaatatctagcctgcagccagaggacttcgccacctactactgtcagcagagccacaacaccccttacaccttcggacagggcaccaagctggaaatcaagcccaaatctagcgacaaaactcacacatgcccaccgtgcccagcacctgaagccgagggggccccgtcagtcttcctcttccccccaaaacccaaggacaccctcatgatctcccggacccctgaggtcacatgcgtggtggtggacgtgagccacgaagaccctgaggtcaagttcaactggtacgtggacggcgtggaggtgcataatgccaagacaaagccgcgggaggagcagtacaacagcacgtaccgtgtggtcagcgtcctcaccgtcctgcaccaggactggctgaatggcaaggagtacaagtgcgccgtctccaacaaagccctcccagcctccatcgagaaaaccatctccaaagccaaagggcagccccgagaaccacaggtgtacaccctgcccccatgccgggaggagatgaccaagaaccaggtcagcctgtggtgcctggtcaaaggcttctatcccagcgacatcgccgtggagtgggagagcaatgggcagccggagaacaactacaagaccacgcctcccgtgctggactccgacggctccttcttcctctatagcgcgctcaccgtggacaagagcaggtggcagcaggggaacgtcttctcatgctccgtgatgcatgaggctctgcacaaccactacacgcagaagagcctctccctgtccccgggtaaatag

SEQ ID NO: 306 - DNA, 1476 bp, synthetic construct
  source 1..1476: mol_type = other DNA; note = GPARC17-scFv-Fc-Hole
atgtacagaatgcagctgctgagctgtatcgccctgtctctggccctggtcaccaactctcagatgcagctggttcagtctggcggcggacttgtgaaacctggcggaagcctgagactgagctgtgccgcttccggcttcaccttcagcagctacaacatgaactgggtccgacaggcccctggcaaaggccttgaatgggtgtccagcatcagcagcagcggcgacttcatgtactacgccgacagcgtgaagggcagattcaccatctccagagacaacgccaagaacagcctgtacctgcagatgagcagcctgagagccgaggataccgccgtgtactactgcgccagagaaggccctggcacaccctttgattattggggccagggcacactggtcaccgtttctagcggaggcggaggatcaggtggtggcggatctggatctacaggctctgccatccagctgacacagagcccttctagcctgtctgccagcgtgggcgacagagtgaccatcacatgtagagccagccagagcatctccagctttctgaactggtatcagcacaagcccggcaaggcccctaagctgctgatctatgtggccagctctctgcagtccggcgtgccatctagattttctggcagcggctccggcaccgacttcaccctgacaatatctagcctgcagccagaggacttcgccacctactactgtcagcagagccacaacaccccttacaccttcggacagggcaccaagctggaaatcaagcccaaatctagcgacaaaactcacacatgcccaccgtgcccagcacctgaagccgagggggccccgtcagtcttcctcttccccccaaaacccaaggacaccctcatgatctcccggacccctgaggtcacatgcgtggtggtggacgtgagccacgaagaccctgaggtcaagttcaactggtacgtggacggcgtggaggtgcataatgccaagacaaagccgcgggaggagcagtacaacagcacgtaccgtgtggtcagcgtcctcaccgtcctgcaccaggactggctgaatggcaaggagtacaagtgcgccgtctccaacaaagccctcccagcctccatcgagaaaaccatctccaaagccaaagggcagccccgagaaccacaggtgtgcaccctgcccccatcccgggaggagatgaccaagaaccaggtcagcctgtcctgcgcggtcaaaggcttctatcccagcgacatcgccgtggagtgggagagcaatgggcagccggagaacaactacaagaccacgcctcccgtgctggactccgacggctccttcaaactcgttagcaagctcaccgtggacaagagcaggtggcagcaggggaacgtcttctcatgctccgtgatgcatgaggctctgcacaaccactacacgcagaagagcctctccctgtccccgggtaaatag

SEQ ID NO: 307 - DNA, 1473 bp, synthetic construct
  source 1..1473: mol_type = other DNA; note = GPARC28-scFv-Fc-Knob
atgtacagaatgcagctgctgagctgtatcgccctgtctctggccctggtcaccaattctgaggtgcagctggtggaatctggcggcggacttgtgaaacctggcggctctctgagactgagctgtgccgcttccggcttcaccttcagcagctacagcatgaactgggtccgacaggcccctggcaaaggccttgaatgggtgtccagcatcagccgggacagcacctacatctactacgccgacagcgtgaagggcagattcaccatctccagagacaacgccaagaacagcctgtacctgcagatgaactccctgagagccgaggacaccgccgtgtactactgtgctagagaaggcgtggcaggcgccttcgatatttggggccagggcacaatggtcaccgtgtctagcggaggcggaggatcaggtggtggtggatctggatctacaggcagcgccatccagctgacacagagccctagtagcctgtctgccagcgtgggcgacagagtgaccatcacatgtagagccagccagagcatcagctcctacctgaactggtatcagcagaagcccggcaaggcccctaagctgctgatctacattgccagcagcctgcagagcggcgtgccaagcagattttctggcagcggctctggcaccgacttcaccctgaccatatctagcctgcagcctgaggacttcgccacctactactgccagcagagctacaacacctggaccttcggacagggcaccaaggtggaaatcaagcccaaatctagcgacaaaactcacacatgcccaccgtgcccagcacctgaagccgagggggccccgtcagtcttcctcttccccccaaaacccaaggacaccctcatgatctcccggacccctgaggtcacatgcgtggtggtggacgtgagccacgaagaccctgaggtcaagttcaactggtacgtggacggcgtggaggtgcataatgccaagacaaagccgcgggaggagcagtacaacagcacgtaccgtgtggtcagcgtcctcaccgtcctgcaccaggactggctgaatggcaaggagtacaagtgcgccgtctccaacaaagccctcccagcctccatcgagaaaaccatctccaaagccaaagggcagccccgagaaccacaggtgtacaccctgcccccatgccgggaggagatgaccaagaaccaggtcagcctgtggtgcctggtcaaaggcttctatcccagcgacatcgccgtggagtgggagagcaatgggcagccggagaacaactacaagaccacgcctcccgtgctggactccgacggctccttcttcctctatagcgcgctcaccgtggacaagagcaggtggcagcaggggaacgtcttctcatgctccgtgatgcatgaggctctgcacaaccactacacgcagaagagcctctccctgtccccgggtaaatag

SEQ ID NO: 308 - DNA, 1473 bp, synthetic construct
  source 1..1473: mol_type = other DNA; note = GPARC28-scFv-Fc-Hole
atgtacagaatgcagctgctgagctgtatcgccctgtctctggccctggtcaccaattctgaggtgcagctggtggaatctggcggcggacttgtgaaacctggcggctctctgagactgagctgtgccgcttccggcttcaccttcagcagctacagcatgaactgggtccgacaggcccctggcaaaggccttgaatgggtgtccagcatcagccgggacagcacctacatctactacgccgacagcgtgaagggcagattcaccatctccagagacaacgccaagaacagcctgtacctgcagatgaactccctgagagccgaggacaccgccgtgtactactgtgctagagaaggcgtggcaggcgccttcgatatttggggccagggcacaatggtcaccgtgtctagcggaggcggaggatcaggtggtggtggatctggatctacaggcagcgccatccagctgacacagagccctagtagcctgtctgccagcgtgggcgacagagtgaccatcacatgtagagccagccagagcatcagctcctacctgaactggtatcagcagaagcccggcaaggcccctaagctgctgatctacattgccagcagcctgcagagcggcgtgccaagcagattttctggcagcggctctggcaccgacttcaccctgaccatatctagcctgcagcctgaggacttcgccacctactactgccagcagagctacaacacctggaccttcggacagggcaccaaggtggaaatcaagcccaaatctagcgacaaaactcacacatgcccaccgtgcccagcacctgaagccgagggggccccgtcagtcttcctcttccccccaaaacccaaggacaccctcatgatctcccggacccctgaggtcacatgcgtggtggtggacgtgagccacgaagaccctgaggtcaagttcaactggtacgtggacggcgtggaggtgcataatgccaagacaaagccgcgggaggagcagtacaacagcacgtaccgtgtggtcagcgtcctcaccgtcctgcaccaggactggctgaatggcaaggagtacaagtgcgccgtctccaacaaagccctcccagcctccatcgagaaaaccatctccaaagccaaagggcagccccgagaaccacaggtgtgcaccctgcccccatcccgggaggagatgaccaagaaccaggtcagcctgtcctgcgcggtcaaaggcttctatcccagcgacatcgccgtggagtgggagagcaatgggcagccggagaacaactacaagaccacgcctcccgtgctggactccgacggctccttcaaactcgttagcaagctcaccgtggacaagagcaggtggcagcaggggaacgtcttctcatgctccgtgatgcatgaggctctgcacaaccactacacgcagaagagcctctccctgtccccgggtaaatag

SEQ ID NO: 309 - protein, 387 aa, synthetic construct
  source 1..387: note = G17-R1CRD-His
MHSSALLCCLVLLTGVRAQMQLVQSGGGLVKPGGSLRLSCAASGFTFSSYNMNWVRQAPGKGLEWVSSISSSGDFMYYADSVKGRFTISRDNAKNSLYLQMSSLRAEDTAVYYCAREGPGTPFDYWGQGTLVTVSSGGGGSGGGGSGSTGSAIQLTQSPSSLSASVGDRVTITCRASQSISSFLNWYQHKPGKAPKLLIYVASSLQSGVPSRFSGSGSGTDFTLTISSLQPEDFATYYCQQSHNTPYTFGQGTKLEIKGGSGGSISAEGSQACAKGCELCSEVNGCLKCSPKLFILLERNDIRQVGVCLPSCPPGYFDARNPDMNKCIKCKIEHCEACFSHNFCTKCKEGLYLHKGRCYPACPEGSSAANGTMECSSPAHHHHHHGA

SEQ ID NO: 310 - protein, 387 aa, synthetic construct
  source 1..387: note = G9-R1CRD-His
MHSSALLCCLVLLTGVRAQVQLVQSGGGLVKPGGSLRLSCAASGFTFSNYNMNWVRQAPGKGLEWVSSISSSGDFMYYADSVKGRFTISRDDAKNSLYLQMNSLRAEDTAVYYCAREGPGTPFDYWGQGTLVTVSSGGGGSGGGGSGSTGSAIQMTQSPSSLSASVGDRVTITCRASQSISSYLNWYQQKPGKAPKLLIYAASSLQSGVPSRFSGSGSGTDFTLTISSLQPEDFATYYCQQSYRTPYTFGQGTKVEIKGGSGGSISAEGSQACAKGCELCSEVNGCLKCSPKLFILLERNDIRQVGVCLPSCPPGYFDARNPDMNKCIKCKIEHCEACFSHNFCTKCKEGLYLHKGRCYPACPEGSSAANGTMECSSPAHHHHHHGA

SEQ ID NO: 311 - protein, 389 aa, synthetic construct
  source 1..389: note = 4D5-R1CRD-His
MHSSALLCCLVLLTGVRAEVQLVESGGGLVQPGGSLRLSCAASGFNIKDTYIHWVRQAPGKGLEWVARIYPTNGYTRYADSVKGRFTISADTSKNTAYLQMNSLRAEDTAVYYCSRWGGDGFYAMDYWGQGTLVTVSSGGGGSGGGGSGGGGSDIQMTQSPSSLSASVGDRVTITCRASQDVNTAVAWYQQKPGKAPKLLIYSASFLYSGVPSRFSGSRSGTDFTLTISSLQPEDFATYYCQQHYTTPPTFGQGTKVEIKGGSGGSISAEGSQACAKGCELCSEVNGCLKCSPKLFILLERNDIRQVGVCLPSCPPGYFDARNPDMNKCIKCKIEHCEACFSHNFCTKCKEGLYLHKGRCYPACPEGSSAANGTMECSSPAHHHHHHGA

SEQ ID NO: 312 - protein, 376 aa, synthetic construct
  source 1..376: note = R1CRD-Fcm
MHSSALLCCLVLLTGVRASRGIKGKRQRRISAEGSQACAKGCELCSEVNGCLKCSPKLFILLERNDIRQVGVCLPSCPPGYFDARNPDMNKCIKCKIEHCEACFSHNFCTKCKEGLYLHKGRCYPACPEGSSAANGTMECSSPAEPKSADKTHTCPPCPAPEAEGAPSVFLFPPKPKDTLMISRTPEVTCVVVDVSHEDPEVKFNWYVDGVEVHNAKTKPREEQYNSTYRVVSVLTVLHQDWLNGKEYKCAVSNKALPASIEKTISKAKGQPREPQVYTLPPSREEMTKNQVSLTCLVKGFYPSDIAVEWESNGQPENNYKTTPPVLDSDGSFFLYSKLTVDKSRWQQGNVFSCSVMHEALHNHYTQKSLSLSPGK

SEQ ID NO: 313 - protein, 389 aa, synthetic construct
  source 1..389: note = R1CRD-GS3-Fcm
MHSSALLCCLVLLTGVRASRGIKGKRQRRISAEGSQACAKGCELCSEVNGCLKCSPKLFILLERNDIRQVGVCLPSCPPGYFDARNPDMNKCIKCKIEHCEACFSHNFCTKCKEGLYLHKGRCYPACPEGSSAANGTMECSSGGGGSGGGGSGGGGSEPKSADKTHTCPPCPAPEAEGAPSVFLFPPKPKDTLMISRTPEVTCVVVDVSHEDPEVKFNWYVDGVEVHNAKTKPREEQYNSTYRVVSVLTVLHQDWLNGKEYKCAVSNKALPASIEKTISKAKGQPREPQVYTLPPSREEMTKNQVSLTCLVKGFYPSDIAVEWESNGQPENNYKTTPPVLDSDGSFFLYSKLTVDKSRWQQGNVFSCSVMHEALHNHYTQKSLSLSPGK

SEQ ID NO: 314 - protein, 371 aa, synthetic construct
  source 1..371: note = R4CRD-GS3-Fcm
MHSSALLCCLVLLTGVRAGGNCTGCIICSEENGCSTCQQRLFLFIRREGIRQYGKCLHDCPPGYFGIRGQEVNRCKKCGATCESCFSQDFCIRCKRQFYLYKGKCLPTCPPGTLAHQNTRECQGGGGGSGGGGSGGGGSEPKSADKTHTCPPCPAPEAEGAPSVFLFPPKPKDTLMISRTPEVTCVVVDVSHEDPEVKFNWYVDGVEVHNAKTKPREEQYNSTYRVVSVLTVLHQDWLNGKEYKCAVSNKALPASIEKTISKAKGQPREPQVYTLPPSREEMTKNQVSLTCLVKGFYPSDIAVEWESNGQPENNYKTTPPVLDSDGSFFLYSKLTVDKSRWQQGNVFSCSVMHEALHNHYTQKSLSLSPGK

SEQ ID NO: 315 - protein, 378 aa, synthetic construct
  source 1..378: note = G17-R4CRD-His
MHSSALLCCLVLLTGVRAQMQLVQSGGGLVKPGGSLRLSCAASGFTFSSYNMNWVRQAPGKGLEWVSSISSSGDFMYYADSVKGRFTISRDNAKNSLYLQMSSLRAEDTAVYYCAREGPGTPFDYWGQGTLVTVSSGGGGSGGGGSGSTGSAIQLTQSPSSLSASVGDRVTITCRASQSISSFLNWYQHKPGKAPKLLIYVASSLQSGVPSRFSGSGSGTDFTLTISSLQPEDFATYYCQQSHNTPYTFGQGTKLEIKGGSGGSGGNCTGCIICSEENGCSTCQQRLFLFIRREGIRQYGKCLHDCPPGYFGIRGQEVNRCKKCGATCESCFSQDFCIRCKRQFYLYKGKCLPTCPPGTLAHQNTRECQGHHHHHHGA

SEQ ID NO: 316 - protein, 378 aa, synthetic construct
  source 1..378: note = G9-R4CRD-His
MHSSALLCCLVLLTGVRAQVQLVQSGGGLVKPGGSLRLSCAASGFTFSNYNMNWVRQAPGKGLEWVSSISSSGDFMYYADSVKGRFTISRDDAKNSLYLQMNSLRAEDTAVYYCAREGPGTPFDYWGQGTLVTVSSGGGGSGGGGSGSTGSAIQMTQSPSSLSASVGDRVTITCRASQSISSYLNWYQQKPGKAPKLLIYAASSLQSGVPSRFSGSGSGTDFTLTISSLQPEDFATYYCQQSYRTPYTFGQGTKVEIKGGSGGSGGNCTGCIICSEENGCSTCQQRLFLFIRREGIRQYGKCLHDCPPGYFGIRGQEVNRCKKCGATCESCFSQDFCIRCKRQFYLYKGKCLPTCPPGTLAHQNTRECQGHHHHHHGA

SEQ ID NO: 317 - protein, 394 aa, synthetic construct
  source 1..394: note = R1CRD-G17-His
MHSSALLCCLVLLTGVRAISAEGSQACAKGCELCSEVNGCLKCSPKLFILLERNDIRQVGVCLPSCPPGYFDARNPDMNKCIKCKIEHCEACFSHNFCTKCKEGLYLHKGRCYPACPEGSSAANGTMECSSGGGGSGGGGSGGGGSQMQLVQSGGGLVKPGGSLRLSCAASGFTFSSYNMNWVRQAPGKGLEWVSSISSSGDFMYYADSVKGRFTISRDNAKNSLYLQMSSLRAEDTAVYYCAREGPGTPFDYWGQGTLVTVSSGGGGSGGGGSGSTGSAIQLTQSPSSLSASVGDRVTITCRASQSISSFLNWYQHKPGKAPKLLIYVASSLQSGVPSRFSGSGSGTDFTLTISSLQPEDFATYYCQQSHNTPYTFGQGTKLEIKHHHHHHGA

SEQ ID NO: 318 - protein, 394 aa, synthetic construct
  source 1..394: note = R1CRD-G9-His
MHSSALLCCLVLLTGVRAISAEGSQACAKGCELCSEVNGCLKCSPKLFILLERNDIRQVGVCLPSCPPGYFDARNPDMNKCIKCKIEHCEACFSHNFCTKCKEGLYLHKGRCYPACPEGSSAANGTMECSSGGGGSGGGGSGGGGSQVQLVQSGGGLVKPGGSLRLSCAASGFTFSNYNMNWVRQAPGKGLEWVSSISSSGDFMYYADSVKGRFTISRDDAKNSLYLQMNSLRAEDTAVYYCAREGPGTPFDYWGQGTLVTVSSGGGGSGGGGSGSTGSAIQMTQSPSSLSASVGDRVTITCRASQSISSYLNWYQQKPGKAPKLLIYAASSLQSGVPSRFSGSGSGTDFTLTISSLQPEDFATYYCQQSYRTPYTFGQGTKVEIKHHHHHHGA

SEQ ID NO: 319 - protein, 624 aa, synthetic construct
  source 1..624: note = G17-R1CRD-GS3-Fcm
MHSSALLCCLVLLTGVRAQMQLVQSGGGLVKPGGSLRLSCAASGFTFSSYNMNWVRQAPGKGLEWVSSISSSGDFMYYADSVKGRFTISRDNAKNSLYLQMSSLRAEDTAVYYCAREGPGTPFDYWGQGTLVTVSSGGGGSGGGGSGSTGSAIQLTQSPSSLSASVGDRVTITCRASQSISSFLNWYQHKPGKAPKLLIYVASSLQSGVPSRFSGSGSGTDFTLTISSLQPEDFATYYCQQSHNTPYTFGQGTKLEIKGGSGGSISAEGSQACAKGCELCSEVNGCLKCSPKLFILLERNDIRQVGVCLPSCPPGYFDARNPDMNKCIKCKIEHCEACFSHNFCTKCKEGLYLHKGRCYPACPEGSSAANGTMECSSGGGGSGGGGSGGGGSEPKSADKTHTCPPCPAPEAEGAPSVFLFPPKPKDTLMISRTPEVTCVVVDVSHEDPEVKFNWYVDGVEVHNAKTKPREEQYNSTYRVVSVLTVLHQDWLNGKEYKCAVSNKALPASIEKTISKAKGQPREPQVYTLPPSREEMTKNQVSLTCLVKGFYPSDIAVEWESNGQPENNYKTTPPVLDSDGSFFLYSKLTVDKSRWQQGNVFSCSVMHEALHNHYTQKSLSLSPGK

SEQ ID NO: 320 - protein, 624 aa, synthetic construct
  source 1..624: note = G9-R1CRD-GS3-Fcm
MHSSALLCCLVLLTGVRAQVQLVQSGGGLVKPGGSLRLSCAASGFTFSNYNMNWVRQAPGKGLEWVSSISSSGDFMYYADSVKGRFTISRDDAKNSLYLQMNSLRAEDTAVYYCAREGPGTPFDYWGQGTLVTVSSGGGGSGGGGSGSTGSAIQMTQSPSSLSASVGDRVTITCRASQSISSYLNWYQQKPGKAPKLLIYAASSLQSGVPSRFSGSGSGTDFTLTISSLQPEDFATYYCQQSYRTPYTFGQGTKVEIKGGSGGSISAEGSQACAKGCELCSEVNGCLKCSPKLFILLERNDIRQVGVCLPSCPPGYFDARNPDMNKCIKCKIEHCEACFSHNFCTKCKEGLYLHKGRCYPACPEGSSAANGTMECSSGGGGSGGGGSGGGGSEPKSADKTHTCPPCPAPEAEGAPSVFLFPPKPKDTLMISRTPEVTCVVVDVSHEDPEVKFNWYVDGVEVHNAKTKPREEQYNSTYRVVSVLTVLHQDWLNGKEYKCAVSNKALPASIEKTISKAKGQPREPQVYTLPPSREEMTKNQVSLTCLVKGFYPSDIAVEWESNGQPENNYKTTPPVLDSDGSFFLYSKLTVDKSRWQQGNVFSCSVMHEALHNHYTQKSLSLSPGK

SEQ ID NO: 321 - protein, 626 aa, synthetic construct
  source 1..626: note = 4D5-R1CRD-GS3-Fcm
MHSSALLCCLVLLTGVRAEVQLVESGGGLVQPGGSLRLSCAASGFNIKDTYIHWVRQAPGKGLEWVARIYPTNGYTRYADSVKGRFTISADTSKNTAYLQMNSLRAEDTAVYYCSRWGGDGFYAMDYWGQGTLVTVSSGGGGSGGGGSGGGGSDIQMTQSPSSLSASVGDRVTITCRASQDVNTAVAWYQQKPGKAPKLLIYSASFLYSGVPSRFSGSRSGTDFTLTISSLQPEDFATYYCQQHYTTPPTFGQGTKVEIKGGSGGSISAEGSQACAKGCELCSEVNGCLKCSPKLFILLERNDIRQVGVCLPSCPPGYFDARNPDMNKCIKCKIEHCEACFSHNFCTKCKEGLYLHKGRCYPACPEGSSAANGTMECSSGGGGSGGGGSGGGGSEPKSADKTHTCPPCPAPEAEGAPSVFLFPPKPKDTLMISRTPEVTCVVVDVSHEDPEVKFNWYVDGVEVHNAKTKPREEQYNSTYRVVSVLTVLHQDWLNGKEYKCAVSNKALPASIEKTISKAKGQPREPQVYTLPPSREEMTKNQVSLTCLVKGFYPSDIAVEWESNGQPENNYKTTPPVLDSDGSFFLYSKLTVDKSRWQQGNVFSCSVMHEALHNHYTQKSLSLSPGK

SEQ ID NO: 322 - protein, 389 aa, synthetic construct
  source 1..389: note = G17-R2CRD-His
MHSSALLCCLVLLTGVRAQMQLVQSGGGLVKPGGSLRLSCAASGFTFSSYNMNWVRQAPGKGLEWVSSISSSGDFMYYADSVKGRFTISRDNAKNSLYLQMSSLRAEDTAVYYCAREGPGTPFDYWGQGTLVTVSSGGGGSGGGGSGSTGSAIQLTQSPSSLSASVGDRVTITCRASQSISSFLNWYQHKPGKAPKLLIYVASSLQSGVPSRFSGSGSGTDFTLTISSLQPEDFATYYCQQSHNTPYTFGQGTKLEIKGGGGSGGGGSGGGGSNPICKGCLSCSKDNGCSRCQQKLFFFLRREGMRQYGECLHSCPSGYYGHRAPDMNRCARCRIENCDSCFSKDFCTKCKVGFYLHRGRCFDECPDGFAPLEETMECVEGHHHHHHGA

SEQ ID NO: 323 - protein, 391 aa, synthetic construct
  source 1..391: note = 4D5-R2CRD-His
MHSSALLCCLVLLTGVRAEVQLVESGGGLVQPGGSLRLSCAASGFNIKDTYIHWVRQAPGKGLEWVARIYPTNGYTRYADSVKGRFTISADTSKNTAYLQMNSLRAEDTAVYYCSRWGGDGFYAMDYWGQGTLVTVSSGGGGSGGGGSGGGGSDIQMTQSPSSLSASVGDRVTITCRASQDVNTAVAWYQQKPGKAPKLLIYSASFLYSGVPSRFSGSRSGTDFTLTISSLQPEDFATYYCQQHYTTPPTFGQGTKVEIKGGGGSGGGGSGGGGSNPICKGCLSCSKDNGCSRCQQKLFFFLRREGMRQYGECLHSCPSGYYGHRAPDMNRCARCRIENCDSCFSKDFCTKCKVGFYLHRGRCFDECPDGFAPLEETMECVEGHHHHHHGA

SEQ ID NO: 324 - protein, 617 aa, synthetic construct
  source 1..617: note = G9-R4CRD-GS3-Fcm
MHSSALLCCLVLLTGVRAQVQLVQSGGGLVKPGGSLRLSCAASGFTFSNYNMNWVRQAPGKGLEWVSSISSSGDFMYYADSVKGRFTISRDDAKNSLYLQMNSLRAEDTAVYYCAREGPGTPFDYWGQGTLVTVSSGGGGSGGGGSGSTGSAIQMTQSPSSLSASVGDRVTITCRASQSISSYLNWYQQKPGKAPKLLIYAASSLQSGVPSRFSGSGSGTDFTLTISSLQPEDFATYYCQQSYRTPYTFGQGTKVEIKGGSGGSGGNCTGCIICSEENGCSTCQQRLFLFIRREGIRQYGKCLHDCPPGYFGIRGQEVNRCKKCGATCESCFSQDFCIRCKRQFYLYKGKCLPTCPPGTLAHQNTRECQGGGGGSGGGGSGGGGSEPKSADKTHTCPPCPAPEAEGAPSVFLFPPKPKDTLMISRTPEVTCVVVDVSHEDPEVKFNWYVDGVEVHNAKTKPREEQYNSTYRVVSVLTVLHQDWLNGKEYKCAVSNKALPASIEKTISKAKGQPREPQVYTLPPSREEMTKNQVSLTCLVKGFYPSDIAVEWESNGQPENNYKTTPPVLDSDGSFFLYSKLTVDKSRWQQGNVFSCSVMHEALHNHYTQKSLSLSPGK

SEQ ID NO: 325 - protein, 619 aa, synthetic construct
  source 1..619: note = 4D5-R4CRD-GS3-Fcm
MHSSALLCCLVLLTGVRAEVQLVESGGGLVQPGGSLRLSCAASGFNIKDTYIHWVRQAPGKGLEWVARIYPTNGYTRYADSVKGRFTISADTSKNTAYLQMNSLRAEDTAVYYCSRWGGDGFYAMDYWGQGTLVTVSSGGGGSGGGGSGGGGSDIQMTQSPSSLSASVGDRVTITCRASQDVNTAVAWYQQKPGKAPKLLIYSASFLYSGVPSRFSGSRSGTDFTLTISSLQPEDFATYYCQQHYTTPPTFGQGTKVEIKGGSGGSGGNCTGCIICSEENGCSTCQQRLFLFIRREGIRQYGKCLHDCPPGYFGIRGQEVNRCKKCGATCESCFSQDFCIRCKRQFYLYKGKCLPTCPPGTLAHQNTRECQGGGGGSGGGGSGGGGSEPKSADKTHTCPPCPAPEAEGAPSVFLFPPKPKDTLMISRTPEVTCVVVDVSHEDPEVKFNWYVDGVEVHNAKTKPREEQYNSTYRVVSVLTVLHQDWLNGKEYKCAVSNKALPASIEKTISKAKGQPREPQVYTLPPSREEMTKNQVSLTCLVKGFYPSDIAVEWESNGQPENNYKTTPPVLDSDGSFFLYSKLTVDKSRWQQGNVFSCSVMHEALHNHYTQKSLSLSPGK

SEQ ID NO: 326 - protein, 319 aa, synthetic construct
  source 1..319: note = G9-R1FU1-His
MHSSALLCCLVLLTGVRAQVQLVQSGGGLVKPGGSLRLSCAASGFTFSNYNMNWVRQAPGKGLEWVSSISSSGDFMYYADSVKGRFTISRDDAKNSLYLQMNSLRAEDTAVYYCAREGPGTPFDYWGQGTLVTVSSGGGGSGGGGSGSTGSAIQMTQSPSSLSASVGDRVTITCRASQSISSYLNWYQQKPGKAPKLLIYAASSLQSGVPSRFSGSGSGTDFTLTISSLQPEDFATYYCQQSYRTPYTFGQGTKVEIKGGSGGSISAEGSQACAKGCELCSEVNGCLKCSPKLFILLERNDIRQVGVCLPSHHHHHHGA

SEQ ID NO: 327 - protein, 382 aa, synthetic construct
  source 1..382: note = G9-R1CRDCys10-His
MHSSALLCCLVLLTGVRAQVQLVQSGGGLVKPGGSLRLSCAASGFTFSNYNMNWVRQAPGKGLEWVSSISSSGDFMYYADSVKGRFTISRDDAKNSLYLQMNSLRAEDTAVYYCAREGPGTPFDYWGQGTLVTVSSGGGGSGGGGSGSTGSAIQMTQSPSSLSASVGDRVTITCRASQSISSYLNWYQQKPGKAPKLLIYAASSLQSGVPSRFSGSGSGTDFTLTISSLQPEDFATYYCQQSYRTPYTFGQGTKVEIKGGSGGSISAEGSQACAKGCELCSEVNGCLKCSPKLFILLERNDIRQVGVCLPSCPPGYFDARNPDMNKCIKCKIEHCEACFSHNFCTKCKEGLYLHKGRCYPACPEGSSAANGTMEHHHHHHGA

SEQ ID NO: 328 - protein, 313 aa, synthetic construct
  source 1..313: note = G9-R2FU1-His
MHSSALLCCLVLLTGVRAQVQLVQSGGGLVKPGGSLRLSCAASGFTFSNYNMNWVRQAPGKGLEWVSSISSSGDFMYYADSVKGRFTISRDDAKNSLYLQMNSLRAEDTAVYYCAREGPGTPFDYWGQGTLVTVSSGGGGSGGGGSGSTGSAIQMTQSPSSLSASVGDRVTITCRASQSISSYLNWYQQKPGKAPKLLIYAASSLQSGVPSRFSGSGSGTDFTLTISSLQPEDFATYYCQQSYRTPYTFGQGTKVEIKGGSGGSNPICKGCLSCSKDNGCSRCQQKLFFFLRREGMRQYGECLHSHHHHHHGA

SEQ ID NO: 329 - protein, 380 aa, synthetic construct
  source 1..380: note = G9-R2CRD-His
MHSSALLCCLVLLTGVRAQVQLVQSGGGLVKPGGSLRLSCAASGFTFSNYNMNWVRQAPGKGLEWVSSISSSGDFMYYADSVKGRFTISRDDAKNSLYLQMNSLRAEDTAVYYCAREGPGTPFDYWGQGTLVTVSSGGGGSGGGGSGSTGSAIQMTQSPSSLSASVGDRVTITCRASQSISSYLNWYQQKPGKAPKLLIYAASSLQSGVPSRFSGSGSGTDFTLTISSLQPEDFATYYCQQSYRTPYTFGQGTKVEIKGGSGGSNPICKGCLSCSKDNGCSRCQQKLFFFLRREGMRQYGECLHSCPSGYYGHRAPDMNRCARCRIENCDSCFSKDFCTKCKVGFYLHRGRCFDECPDGFAPLEETMECVEGHHHHHHGA

SEQ ID NO: 330 - protein, 240 aa, synthetic construct; identical to SEQ ID NO: 21
  source 1..240: note = G17

SEQ ID NO: 331 - protein, 240 aa, synthetic construct; identical to SEQ ID NO: 20
  source 1..240: note = G9

SEQ ID NO: 332 - protein, 242 aa, synthetic construct
  source 1..242: note = 4D5
EVQLVESGGGLVQPGGSLRLSCAASGFNIKDTYIHWVRQAPGKGLEWVARIYPTNGYTRYADSVKGRFTISADTSKNTAYLQMNSLRAEDTAVYYCSRWGGDGFYAMDYWGQGTLVTVSSGGGGSGGGGSGGGGSDIQMTQSPSSLSASVGDRVTITCRASQDVNTAVAWYQQKPGKAPKLLIYSASFLYSGVPSRFSGSRSGTDFTLTISSLQPEDFATYYCQQHYTTPPTFGQGTKVEIK

SEQ ID NO: 333 - protein, 113 aa, synthetic construct
  source 1..113: note = R1CRD
ISAEGSQACAKGCELCSEVNGCLKCSPKLFILLERNDIRQVGVCLPSCPPGYFDARNPDMNKCIKCKIEHCEACFSHNFCTKCKEGLYLHKGRCYPACPEGSSAANGTMECSS

SEQ ID NO: 334 - protein, 104 aa, synthetic construct
  source 1..104: note = R4CRD
NCTGCIICSEENGCSTCQQRLFLFIRREGIRQYGKCLHDCPPGYFGIRGQEVNRCKKCGATCESCFSQDFCIRCKRQFYLYKGKCLPTCPPGTLAHQNTRECQG

SEQ ID NO: 335 - protein, 108 aa, synthetic construct
  source 1..108: note = R2CRD
NPICKGCLSCSKDNGCSRCQQKLFFFLRREGMRQYGECLHSCPSGYYGHRAPDMNRCARCRIENCDSCFSKDFCTKCKVGFYLHRGRCFDECPDGFAPLEETMECVEG

SEQ ID NO: 336 - protein, 47 aa, synthetic construct
  source 1..47: note = R1FU1
ISAEGSQACAKGCELCSEVNGCLKCSPKLFILLERNDIRQVGVCLPS

SEQ ID NO: 337 - protein, 110 aa, synthetic construct
  source 1..110: note = R1CRDCys10
ISAEGSQACAKGCELCSEVNGCLKCSPKLFILLERNDIRQVGVCLPSCPPGYFDARNPDMNKCIKCKIEHCEACFSHNFCTKCKEGLYLHKGRCYPACPEGSSAANGTME

SEQ ID NO: 338 - protein, 41 aa, synthetic construct
  source 1..41: note = R2FU1
NPICKGCLSCSKDNGCSRCQQKLFFFLRREGMRQYGECLHS

SEQ ID NO: 339 - protein, 8 aa, synthetic construct
  source 1..8: note = His
HHHHHHGA

SEQ ID NO: 340 - protein, 234 aa, synthetic construct
  source 1..234: note = Fcm
PAEPKSADKTHTCPPCPAPEAEGAPSVFLFPPKPKDTLMISRTPEVTCVVVDVSHEDPEVKFNWYVDGVEVHNAKTKPREEQYNSTYRVVSVLTVLHQDWLNGKEYKCAVSNKALPASIEKTISKAKGQPREPQVYTLPPSREEMTKNQVSLTCLVKGFYPSDIAVEWESNGQPENNYKTTPPVLDSDGSFFLYSKLTVDKSRWQQGNVFSCSVMHEALHNHYTQKSLSLSPGK

SEQ ID NO: 341 - protein, 247 aa, synthetic construct
  source 1..247: note = GS3 linker-Fcm
GGGGSGGGGSGGGGSEPKSADKTHTCPPCPAPEAEGAPSVFLFPPKPKDTLMISRTPEVTCVVVDVSHEDPEVKFNWYVDGVEVHNAKTKPREEQYNSTYRVVSVLTVLHQDWLNGKEYKCAVSNKALPASIEKTISKAKGQPREPQVYTLPPSREEMTKNQVSLTCLVKGFYPSDIAVEWESNGQPENNYKTTPPVLDSDGSFFLYSKLTVDKSRWQQGNVFSCSVMHEALHNHYTQKSLSLSPGK

SEQ ID NO: 342 - protein, 18 aa, synthetic construct
  source 1..18: note = hIL-10ss
MHSSALLCCLVLLTGVRA

SEQ ID NO: 343 - protein, 262 aa, synthetic construct
  source 1..262: note = G17:GPA33_2R_C17_scFv-His
QMQLVQSGGGLVKPGGSLRLSCAASGFTFSSYNMNWVRQAPGKGLEWVSSISSSGDFMYYADSVKGRFTISRDNAKNSLYLQMSSLRAEDTAVYYCAREGPGTPFDYWGQGTLVTVSSGGGGSGGGGSGSTGSAIQLTQSPSSLSASVGDRVTITCRASQSISSFLNWYQHKPGKAPKLLIYVASSLQSGVPSRFSGSGSGTDFTLTISSLQPEDFATYYCQQSHNTPYTFGQGTKLEIKEPRTPRPCLVPRGSHHHHHHGA

SEQ ID NO: 344 - protein, 262 aa, synthetic construct
  source 1..262: note = G9:GPA33_2R_C9_scFv-His
QVQLVQSGGGLVKPGGSLRLSCAASGFTFSNYNMNWVRQAPGKGLEWVSSISSSGDFMYYADSVKGRFTISRDDAKNSLYLQMNSLRAEDTAVYYCAREGPGTPFDYWGQGTLVTVSSGGGGSGGGGSGSTGSAIQMTQSPSSLSASVGDRVTITCRASQSISSYLNWYQQKPGKAPKLLIYAASSLQSGVPSRFSGSGSGTDFTLTISSLQPEDFATYYCQQSYRTPYTFGQGTKVEIKEPRTPRPCLVPRGSHHHHHHGA

SEQ ID NO: 345 - protein, 264 aa, synthetic construct
  source 1..264: note = 4D5_scFv-His
EVQLVESGGGLVQPGGSLRLSCAASGFNIKDTYIHWVRQAPGKGLEWVARIYPTNGYTRYADSVKGRFTISADTSKNTAYLQMNSLRAEDTAVYYCSRWGGDGFYAMDYWGQGTLVTVSSGGGGSGGGGSGGGGSDIQMTQSPSSLSASVGDRVTITCRASQDVNTAVAWYQQKPGKAPKLLIYSASFLYSGVPSRFSGSRSGTDFTLTISSLQPEDFATYYCQQHYTTPPTFGQGTKVEIKEPRTPRPCLVPRGSHHHHHHGA

SEQ ID NO: 346 - protein, 551 aa, synthetic construct
  source 1..551: note = G17-mG2aFc-PDGFTM
MYRMQLLSCIALSLALVTNSQMQLVQSGGGLVKPGGSLRLSCAASGFTFSSYNMNWVRQAPGKGLEWVSSISSSGDFMYYADSVKGRFTISRDNAKNSLYLQMSSLRAEDTAVYYCAREGPGTPFDYWGQGTLVTVSSGGGGSGGGGSGSTGSAIQLTQSPSSLSASVGDRVTITCRASQSISSFLNWYQHKPGKAPKLLIYVASSLQSGVPSRFSGSGSGTDFTLTISSLQPEDFATYYCQQSHNTPYTFGQGTKLEIKPKSSDPRGPTIKPCPPCKCPAPNLLGGPSVFIFPPKIKDVLMISLSPIVTCVVVDVSEDDPDVQISWFVNNVEVHTAQTQTHREDYNSTLRVVSALPIQHQDWMSGKEFKCKVNNKDLPAPIERTISKPKGSVRAPQVYVLPPPEEEMTKKQVTLTCMVTDFMPEDIYVEWTNNGKTELNYKNTEPVLDSDGSYFMYSKLRVEKKNWVERNSYSCSVVHEGLHNHHTTKSFSRTPGKGGSGNAVGQDTQEVIVVPHSLPFKVVVISAILALVVLTIISLIILIMLWQKKPR

SEQ ID NO: 347 - protein, 545 aa, synthetic construct
  source 1..545: note = G17-Fcwt-PDGFTM
MYRMQLLSCIALSLALVTNSQMQLVQSGGGLVKPGGSLRLSCAASGFTFSSYNMNWVRQAPGKGLEWVSSISSSGDFMYYADSVKGRFTISRDNAKNSLYLQMSSLRAEDTAVYYCAREGPGTPFDYWGQGTLVTVSSGGGGSGGGGSGSTGSAIQLTQSPSSLSASVGDRVTITCRASQSISSFLNWYQHKPGKAPKLLIYVASSLQSGVPSRFSGSGSGTDFTLTISSLQPEDFATYYCQQSHNTPYTFGQGTKLEIKPKSSDKTHTCPPCPAPELLGGPSVFLFPPKPKDTLMISRTPEVTCVVVDVSHEDPEVKFNWYVDGVEVHNAKTKPREEQYNSTYRVVSVLTVLHQDWLNGKEYKCKVSNKALPAPIEKTISKAKGQPREPQVYTLPPSRDELTKNQVSLTCLVKGFYPSDIAVEWESNGQPENNYKTTPPVLDSDGSFFLYSKLTVDKSRWQQGNVFSCSVMHEALHNHYTQKSLSLSPGKGGSGNAVGQDTQEVIVVPHSLPFKVVVISAILALVVLTIISLIILIMLWQKKPR

SEQ ID NO: 348 - protein, 545 aa, synthetic construct
  source 1..545: note = G9-Fcm-PDGFTM
MYRMQLLSCIALSLALVTNSQVQLVQSGGGLVKPGGSLRLSCAASGFTFSNYNMNWVRQAPGKGLEWVSSISSSGDFMYYADSVKGRFTISRDDAKNSLYLQMNSLRAEDTAVYYCAREGPGTPFDYWGQGTLVTVSSGGGGSGGGGSGSTGSAIQMTQSPSSLSASVGDRVTITCRASQSISSYLNWYQQKPGKAPKLLIYAASSLQSGVPSRFSGSGSGTDFTLTISSLQPEDFATYYCQQSYRTPYTFGQGTKVEIKPKSSDKTHTCPPCPAPEAEGAPSVFLFPPKPKDTLMISRTPEVTCVVVDVSHEDPEVKFNWYVDGVEVHNAKTKPREEQYNSTYRVVSVLTVLHQDWLNGKEYKCAVSNKALPASIEKTISKAKGQPREPQVYTLPPSREEMTKNQVSLTCLVKGFYPSDIAVEWESNGQPENNYKTTPPVLDSDGSFFLYSKLTVDKSRWQQGNVFSCSVMHEALHNHYTQKSLSLSPGKGGSGNAVGQDTQEVIVVPHSLPFKVVVISAILALVVLTIISLIILIMLWQKKPR

SEQ ID NO: 349 - protein, 547 aa, synthetic construct
  source 1..547: note = 4D5-Fcm-PDGFTM
MYRMQLLSCIALSLALVTNSEVQLVESGGGLVQPGGSLRLSCAASGFNIKDTYIHWVRQAPGKGLEWVARIYPTNGYTRYADSVKGRFTISADTSKNTAYLQMNSLRAEDTAVYYCSRWGGDGFYAMDYWGQGTLVTVSSGGGGSGGGGSGGGGSDIQMTQSPSSLSASVGDRVTITCRASQDVNTAVAWYQQKPGKAPKLLIYSASFLYSGVPSRFSGSRSGTDFTLTISSLQPEDFATYYCQQHYTTPPTFGQGTKVEIKPKSSDKTHTCPPCPAPEAEGAPSVFLFPPKPKDTLMISRTPEVTCVVVDVSHEDPEVKFNWYVDGVEVHNAKTKPREEQYNSTYRVVSVLTVLHQDWLNGKEYKCAVSNKALPASIEKTISKAKGQPREPQVYTLPPSREEMTKNQVSLTCLVKGFYPSDIAVEWESNGQPENNYKTTPPVLDSDGSFFLYSKLTVDKSRWQQGNVFSCSVMHEALHNHYTQKSLSLSPGKGGSGNAVGQDTQEVIVVPHSLPFKVVVISAILALVVLTIISLIILIMLWQKKPR

SEQ ID NO: 350 - protein, 237 aa, synthetic construct
  source 1..237: note = mG2aFc
PKSSDPRGPTIKPCPPCKCPAPNLLGGPSVFIFPPKIKDVLMISLSPIVTCVVVDVSEDDPDVQISWFVNNVEVHTAQTQTHREDYNSTLRVVSALPIQHQDWMSGKEFKCKVNNKDLPAPIERTISKPKGSVRAPQVYVLPPPEEEMTKKQVTLTCMVTDFMPEDIYVEWTNNGKTELNYKNTEPVLDSDGSYFMYSKLRVEKKNWVERNSYSCSVVHEGLHNHHTTKSFSRTPGK

SEQ ID NO: 351 - protein, 231 aa, synthetic construct
  source 1..231: note = Fcwt
PKSSDKTHTCPPCPAPELLGGPSVFLFPPKPKDTLMISRTPEVTCVVVDVSHEDPEVKFNWYVDGVEVHNAKTKPREEQYNSTYRVVSVLTVLHQDWLNGKEYKCKVSNKALPAPIEKTISKAKGQPREPQVYTLPPSRDELTKNQVSLTCLVKGFYPSDIAVEWESNGQPENNYKTTPPVLDSDGSFFLYSKLTVDKSRWQQGNVFSCSVMHEALHNHYTQKSLSLSPGK

SEQ ID NO: 352 - protein, 54 aa, synthetic construct
  source 1..54: note = PDGFTM
GGSGNAVGQDTQEVIVVPHSLPFKVVVISAILALVVLTIISLIILIMLWQKKPR

SEQ ID NO: 353 - protein, 20 aa, synthetic construct
  source 1..20: note = hIL-2ss
MYRMQLLSCIALSLALVTNS